European Patent Application EP 4 707 388 A1, published March 11, 2026. Title: BIOENZYME FOR CATALYZING FORMATION OF THREE-MEMBERED OR FOUR-MEMBERED OXYGEN HETEROCYCLIC STRUCTURE OF TAXANE MOLECULE, AND GENE, BIOMATERIAL AND USE THEREOF. Applicant: Agricultural Genomics Institute at Shenzhen, Chinese Academy of Agricultural Sciences; Shenzhen Branch, Guangdong Laboratory for Lingnan Modern Agriculture. The sequence listing filed with the application follows.

SEQUENCE LISTING (164 sequences)

SEQ ID NO: 1 - DNA, 1524 bp, unidentified
  source 1..1524: mol_type = other DNA; note = TOT reference gene; note (original language) = TOT参考基因
atggttcatgtgttgcaggtagtgaaaatggatagagttagagaaatatttaatggaagttcaggttctccagctggtattccccacagtgtgatcacagccggtgtgggtgccataataataattcttctgtcactactgctcctccgccgttctagtaaacggggcgactcctctcatcctcctgggaattcaggccttccattcattggagagacattatcattcaccaaggcttttaaatcgaacacgctggccgaattttttgaggagagggtgaagaaattcgggaatgtatttaagatttcaataatcgggcctcccacagtggtaatgtgcggcaatgagggaaaccggtttattttcgccaacgaggagaagcttgtccacttgtcgtggtctggtcgatatgcgaaaatcctgggtggagattccgtttccatgaagaggggagatgatcatcgcagtgtacgtgccgcattcgcagggtttttgagccctgcatcgctgcctatttacataagtaaaatgagtgcacagatccaagatcatatcaaccaaaaatggaaaggaaaagatgtaattgctgtagttcctctggtaaaggagctcgtcttcaacgtttcctacaacttgtttttcagcataaatgatagcgaggaactgcatcgattgcataagattttcgaaactattgtggagggacatgtttccatgccgatagaccttcccggattcacctttcatagagcacttcagggaagggcgaagctcaagaaagttttctcttctttaatagaaaggagaagaagcgatctgagctccggattggcatctgctaatcaggatctcatctctgttttactcacctacaaagatgatagggggtatacaatgacccacgacgagctcctcgacaactttctttcccttcttgaatcctcctatgattccgtcaattcaccaatggcctgcatttttaagcttttgtatgccaatccagaatgctatgaaaaagtagttcaagagcaattggggatactttctggtaagaaggaaggacaagaaatctcgtggaaggatctgagatccatgaaatacacatggcaagtacttcaggaaacgctacgactgtatactcaagttgctggaatatttcgcaaagccatgactgtcattcattatgatggtcacaccattcccaaagggtggcaacttctttgggcaacccaaactacacatctgaacgacaaatatttcagtgagccggaaaaattcatgccttccagattcgatgaagaaggaaacaatgtgattccttactcattcgtaccatttggaggagggcggcggatgtgtccaggttgggaattcggaaagatggagatcttactcttcgtccatcactttgttaaagcgttcagtggctttaccccaatcgatccggacgaaaaaattactgggaatccatttcctcatctccctgccaatggattttcaataaaacctactcccagatcctaa

SEQ ID NO: 2 - DNA, 1524 bp, unidentified
  source 1..1524: mol_type = other DNA; note = TOT homologous gene; note (original language) = TOT同源基因
atggttcatgtgttgcaggtagtgaaaatggatagagttagtgaaatatttaatggaagttcaggttctccagctggtattccccacagtgtgatcacagccggtgtgggtgccataataataattcttctgtcactagtgctcctccgccgttctagtaaacggggcgactcctctcatcctcctgggaattcaggccttccattcattggggagacattatcattcaccaaggcttttaaatcgaacacgctggccgaattttttgaggagagggtgaagaaattcgggaatgtatttaagatttcaataatcgggcctcccacagtggtaatgtgcggcaatgagggaaaccggtttattttcgccaacgaggagaagctgatgcacctgtcgtggtccggtcggtatgcgaaaatccttggtggggaatccgtttccatgaagaggggagatgatcatcgcagtgtacgtgccgcattcgcagggtttttgagcccttcggcgctgcctctttacgtagctaaaatgagtgcgcagatccaaaatcatatcaacgagaaatggaaaggaagagatgtaattgctgtagttcctttggtaaaagagctggtcttcaacgtttcctccaacttgtttttcagcatgaatgatagcgaggaattgcatcgattgcatcaaattttcgaaactattgtagatggacatgtttccatgccgatagaccttcccggattcacctttcataaagcacttcagggaagggcgaagctcaagaaagtttactcttctttaatagaaaggagaagaagcgatctgagctccggattggcatctgctaatcaggatctcatctctgttttactcacctacaaagatgatagggggtatacaatgacccacgacgagctcctcgacaattttctttcccttattgaatcctcctatgattccatcaattcaccaatggcctgcatttttaagcttttgtatgccaatccagaatgctatgaaaaagtagttcaagagcaattggggatactttctggtaagaaggaaggagaagaaatctcatggaaggatctgagatccatgaaatacacatggcaagcaattcaggaaacgctacgaatttatactcaagttgcaggaatatttcgcaaagccatgactgacattcattatgatggtcacaccattcccaaagggtggcaacttctttgggcaacccaaactacacatctgaacgacaaatatttcagtgagcctgaaaaattcatgccttccagattcgatgaagaaggaaacaatgtgattccttactcattcgtaccatttggaggagggcggcggatgtgtccaggttgggaattcggaaagatggagatcttactctttgtccatcactttgttaaaacgttcagtggctttaccccaattgatccgaacgaaaaaattactgggaatccttttcctcatctccctgccaatggatttctaataaaacctattctcagatcctaa

SEQ ID NO: 3 - DNA, 1524 bp, unidentified
  source 1..1524: mol_type = other DNA; note = TOT homologous gene; note (original language) = TOT同源基因
atggttcatgtgttgcacgtagtgaaaatggatagagttagagaaatatttaatggaagttcaggttctccagctggtattccccacagtgtgatcacagccggtgtgggtgccataataataattcttctgtcactactgctcctccgccgttctagtaaacggggcgactcctctcatcctcctgggaattcaggccttccattcattggggagacattatcattcaccaaggcttttaaatcgaacacgctggccgaattttttgaggagagggtgaagaaattcgggaatgtatttaagatttcaataatcgggcctcccacagtggtaatgtgcggcaatgagggaaaccggtttattttcgccaacgaggagaagctgatgcacctgtcgtggtccggtcgatatgcgaaaatccttggtggggaatccgtttccatgaagaggggagatgatcatcgcagtgtacgtgccgcattcgcagggtttttgagctctgcatcgctgcctgtttacataagtaaaatgagtgcacagatccaagatcatatcaacgaaaaatggaaaggaaaagatgtaattgctgtagttcctctggtaaaggagctcgtcttcaacgtttcctacaacttgtttttcagcataaatgatagcgaggaactgcatcgattgcataagattttcgaaactattgtggagggacatctttccatgccgatagaccttcccggattcacctttcatagagcacttcagggaagggcgaagctcaagaaagttttctcttctttaatagaaaggagaagaagcgatctgagctccggattggcatctgctaatcaggatctcatttctgttttactcacctacaaagatgatagggggtatacaatgacccacgacgagctcctcgacaactttctttcccttcttgaaggctcctatgattccatcaattcaccaatggcctgcatttttaagcttttgtatgacaatccagaatgctatgaaaaagtagttcaagagcaattggggatactttctggtaagaaggaaggacaagaaatctcgtggaaggatctgagatccatgaaatacacatggcaagtacttcaggaaacgctacgactgtatactcaagttgctggaatatttcgcaaagccatgactgacattcattatgatggtcacaccattcccaaagggtggcaacttctttgggcaaaccaaactacacatctgaacgacaaatatttcagtgagcctgaaaaattcatgccttccagattcgatgaagaaggaaacaatatgattccttactcattcgtaccatttggaggagggcggcggatgtgtccaggttgggaattcggaaagatggagatcttactctttgtccatcactttgttaaaacgttcagtggctttaccccaattgatccgaacgaaaaaattactgggaatccttttcctcatctccctgccaatggatttctaataaaacctattctcagatcctaa

SEQ ID NO: 4 - DNA, 1524 bp, unidentified
  source 1..1524: mol_type = other DNA; note = TOT homologous gene; note (original language) = TOT同源基因
atggttcatgtgttgcaggtagtgaaaatggatagagttagtgaaatatttaatggaagttcaggttctccagctggtattccccacagtgtgatcacagccggtgtgggtgccataataataattcttctgtcactagtgctcctccgccgttctagtaaacggggcgactcctctcatcctcctgggaattcaggccttccattcattggggagacattatcattcaccaaggcttttaaatcgaacacgctggccgaattttttgaggagagggtgaagaaattcgggaatgtatttaagatttcaataatcgggcctcccacagtggtaatgtgcggcaatgagggaaaccggtttattttcgccaacgaggagaagctgatgcacctgtcgtggtccggtcggtatgcgaaaatccttggtggggaatccgtttccatgaagaggggagatgatcatcgcagtgtacgtgccgcattcgcagggtttttgagcccttcggcgctgcctctttacgtagctaaaatgagtgcgcagatccaaaatcatatcaacgagaaatggaaaggaagagatgtaattgctgtagttcctttggtaaaagagctggtcttcaacgtttcctccaacttgtttttcagcatgaatgatagcgaggaattgcatcgattgcatcaaattttcgaaactattgtagatggacatgtttccatgccgatagaccttcccggattcacctttcataaagcacttcagggaagggcgaagctcaagaaagtttactcttctttaatagaaaggagaagaagcgatctgagctccggattggcatctgctaatcaggatctcatctctgttttactcacctacaaagatgatagggggtatacaatgacccacgacgagctcctcgacaattttctttcccttattgaatcctcctatgattccgtcaattcaccaatggcctgcatttttaagcttttgtatgccaatccagaatgctatgaaaaagtagttcaagagcaattggggatactttctggtaagaaggaaggacaagaaatctcgtggaaggatctgagatccatgaaatacacatggcaagtacttcaggaaacgctacgactgtatactcaagttgctggaatatttcgcaaagccatgactgtcattcattatgatggtcacaccattcccaaagggtggcaacttctttgggcaacccaaactacacatctgaacgacaaatatttcagtgagccgcaaaaattcatgccttccagattcgatgaagaaggaaacaatgtgattccttactcattcgtaccatttggaggagggcggcggatgtgtccaggttgggaattcggaaagatggagatcttactcttcgtccatcactttgttaaagcgttcagtggctttaccccaatcgatccggacgaaaaaattactgggaatccttttcctcatctccctgccaatggatttctaataaaacctattctcagatcctaa

SEQ ID NO: 5 - DNA, 1482 bp, unidentified
  source 1..1482: mol_type = other DNA; note = TOT homologous gene; note (original language) = TOT同源基因
atggatacagttagagaattgaatggaggatcaggttcctctggtattcccctcagtctgatcaccgccgctgtgggtgccataataattctgtcactactgctcctccgccgttctaaacggggcaactcatctcatcctcctgggaattcagggcttccattcattggggagacattatcattcaccaaggcttttaaatcgaacacgctggaccaattttttgaggagagggtgaagaaattcgggcaagtctttaagctttccgtaatcgggcctcccacagtggcaatgtgcggccctgagggaaaccggtttgttttcgccaacgaggagaagcttgtccacttgtcgtggtctggtcgatatgcgaaaatcctgggtggagattccgtttccatgaagaggggagatgatcatcgcagtgtacgtgccgcattcgcagggtttttgagccctgcatcgctgcctgtttacataagtaaaatgagtgcacagatccaagatcatatcaacgaaaaatggaaaggaaaagatgtaattgctgtagttcctctggtaaaggagctcgtcttcaacgtttcctacaacttgtttttcagcataaatgatagcgaggaactgcatcgattgcataagattttcgaaactattgtggagggacatgtttccatgccgatagaccttcccggattcacctttcatagagcacttcagggaagggcgaagctcaagaaagttttctcttctttaatagaaaggagaagaagcgatcttagctccggattggcatctgctaatcaggatctcatttctgttttactcacctacaaagatgatagggggtatacaatgacccacgacgagctcctcgacaactttctttcccttcttgaagcctcctatgattccgtcaattcaccaatggcctgcatttttaagcttttgtatgccaatccagaatgctatgaaaaagtagttcaagagcaattggggatactttctggtaagaaggaaggacaagaaatctcgtggaaggatctgagatccatgaaatacacatggcaagtacttcaggaaacgctacgactgtatactcaagttgctggaatatttcgcaaagccatgactgacattcattataatggtcataccattcccaaagggtggcaacttctttgggcaacccaaactacacatctgaacgacaaatatttcagtgagccggaaaaattcatgccttccagattcgatgaagaaggaaacaatgtgattccttactcattcgtaccatttggaggagggcggcggatgtgtccaggttgggaattcggaaagatggagatcttactcttcgtccatcactttgttaaagcgttcagtggctttaccccaatcgatccggacgaaaaaattactgggaatccatttcctcatctccctgccaatggattttcaataaaacctactcccagatcctaa

SEQ ID NO: 6 - DNA, 1524 bp, unidentified
  source 1..1524: mol_type = other DNA; note = TOT homologous gene; note (original language) = TOT同源基因
atggttcatgtgttgcaggtagtgaaaatggatagagttagtgaaatatttaatggaagttcaggttctccagctggtattccccacagtgtgatcacagccggtgtgggtgccataataataattcttctgtcactagtgctcctccgccgttctagtaaacggggcgactcctctcatcctcctgggaattcaggccttccattcattggggagacattatcattcaccaaggcttttaaatcgaacacgctggccgaattttttgaggagagggtgaagaaattcgggaatgtatttaagatttcaataatcgggcctcccacagtggtaatgtgcggcaatgagggaaaccggtttattttcgccaacgaggagaagctgatgcacctgtcgtggtccggtcgatatgcgaaaatccttggtggggaatccgtttccatgaagaggggagatgatcatcgcagtgtacgtgccgcattcgcagggtttttgagcccttcggcgctgcctctttacgtagctaaaatgagtgcgcagatccaaaatcatatcaacgagaaatggaaaggaagagatgtaattgctgtagttcctttggtaaaagagctggtcttcaacgtttcctccaacttgtttttcggcatgaatgatagcgaggaactgcatcgattgcatcaaattttcgaaactattgtagatggacatgtttccatgccgatagaccttcccggattcacctttcataaagcacttcagggaagggcgaagctcaagaaagtttactcttctttaatagaaaggagaagaagcgatctgagctccggattggcatctgctaatcaggatctcatctctgttttactcacctacaaagatgatagggggtatacaatgacccacgtcgagctcctcgacaattttctttcccttattgaatcctcctatgattccatcaattcaccaatggcctgcatttttaagcttttgtatgccaatccagaatgctatgaaaaagtagttcaagagcaattggggatactctctggtaagaaggaaggagaagaaatctcatggaaggatctgagatccatgaaatacacatggcaagcaattcaggaaacgctacgaatttatactcaagttgcaggaatatttcgcaaagccatgactgacattcattatgatggtcacaccattcccaaagggtggcaacttctttgggcaacccaaactacacatctgaacgacaaatatttcagtgagcctgaaaaattcatgccttccagattcgatgaagaaggaaacaatgtgattccttactcattcgtaccatttggaggagggcggcggatgtgtccaggttgggaattcggaaagatggagatcttactctttgtccatcactttgttaaaacgttcagtggctttaccccaattgatccgaacgaaaaaattactgggaatccttttcctcatctccctgccaatggatttctaataaaacctattctcagatcctaa

SEQ ID NO: 7 - DNA, 1524 bp, unidentified
  source 1..1524: mol_type = other DNA; note = TOT homologous gene; note (original language) = TOT同源基因
atggttcatgtgttgcaggtagtgaaaatgtatagagttagtgaaatatttaatggaagttcaggttctccagctggtattccccacagtgtgatcacagccggtgtgggtgccataataataattcttctgtcactagtgctcctccgccgttctagtaaacggggcgactcctctcatcctcctgggaattcaggccttccattcattggggagacattatcattcaccaaggcttttaaatcgaacacgctggccgaattttttgaggagagggtgaagaaattcgggaatgtatttaagatttcaataatcgggcctcccacagtggtaatgtgcggcaatgagggaaaccggtttattttcgccaacgaggagaagctgatgcacctgtcgtggtccggtcggtatgcgaaaatccttggtggggaatccgtttccatgaagaggggagatgatcatcgcagtgtacgtgccgcattcgcagggtttttgagcccttcggcgctgcctctttacgtagctaaaatgagtgcgcagatccaaaatcatatcaacgagaaatggaaaggaagagatgtaattgctgtagttcctttggtaaaagagctggtcttcaacgtttcctccaacttgtttttcagcatgaatgatagcgaggaattgcatcgattgcatcaaattttcgaaactattgtagatggacatgtttccatgccgatagaccttcccggattcacctttcataaagcacttcagggaagggcgaagctcaagaaagtttactcttctttaatagaaaggagaagaagcgatctgagctccggattggcatctgctaatcaggatctcatctctgttttactcacctacaaagatgatagggggtatacaatgacccacgacgagctcctcgacaattttctttcccttattgaatcctcctatgattccatcaattcaccaatggcctgcatttttaagcttttgtatgccaatccagaatgctatgaaaaagtagttcaagagcaattggggatactttctggtaagaaggaaggagaagaaatctcatggaaggatctgagatccatgaaatacacatggcaagcaattcaggaaacgctacgaatttatactcaagttgcaggaatatttcgcaaagccatgactgacattcattatgatggtcacaccattcccaaagggtggcaacttctttgggcaacccaaactacacatctgaacgacaaatatttcagtgagcctgaaaaattcatgccttccagattcgatgaagaaggaaacaatgtgattccttactcattcgtaccatttggaggagggcggcggatgtgtccaggttgggaattcggaaagatggagatcttactctttgtccatcactttgttaaaacgttcagtggctttaccccaattgatccgaacgaaaaaattactgggaatccttttcctcatctccctgccaatggatttctaataaaacctattctcagatcctaa

SEQ ID NO: 8 - DNA, 1482 bp, unidentified
  source 1..1482: mol_type = other DNA; note = TOT homologous gene; note (original language) = TOT同源基因
atggatacagttagagaattgaatggaggatcaggttcccctggtattcccctcagtctgatcaccgccgctgtgggtgccataataattctgtcactactgctcctccgccgttctaaacggggcaactcatctcatcctcctgggaattcagggcttccattcattggggagacattatcattcaccaaggcttttaaatcgaacacgctggaccaattttttgaggagagggtgaagaaattcgggcaagtctttaagctttccgtaatcgggcctcccacagtggcaatgtgcggccctgagggaaaccggtttgttttcgccaacgaggagaagcttgtccacttgtcgtggtctggtcgatatgcgaaaatcctgggtggagattccgtttccatgaagaggggagatgatcatcgcagagtacgtgccgcattcgcagggtttttgagccctgcatcactgcctgtttacataagtaaaatgagtgcacagatccaagatcatatcaacgaaaaatggaaagaaaaagttgtaattgctgtagttcctctggtaaaggagctcgtcttcaacgtttcctacaacttgtttttcagcataaatgatagcgaggaactgcatcgattgcataagattttcgaaactattgtggagggacatgtttccatgccgatagaccttcccggattcacctttcatagagcacttcagggaagggcgaagctcaagaaagttttctcttctttaatagaaaggagaagaagcgatctgagctccggattggcatctgctaatcaggatctcatctctgttttactcacctacaaagatgatagggggtatacaatgacccacgacgagctcctcgacaactttctttcccttcttgaatcctcctatgattccgtcaattcaccaatggcctgcatttttaagcttttgtatgacaatccagaatgctatgaaaaagtagttcaagagcaattggggatactttctggtaagaaggaaggacaagaaatctcgtggaaggatctgagatccatgaaatacacatggcaagtacttcaggaaacgctacgactgtatactcaagttgctggaatatttcgcaaagccatgactgacattcattatgatggtcacaccattcccaaagggtggcaacttctttgggcaacccaaactacacatctgaacgacaaatatttcagtgagccggaaaagttcatgccttccagattcgatgaagaaggaaacaatttgattccttactcattcgtaccatttggaggagggcggcggatgtgtccaggttgggaattcggaaagatggagatcttactcttcgtccatcactttgttaaagcgttcagtggctttaccccaatcgatccggacgaaaaaattactgggaatccatttcctcatctccctgccaatggattttcaataaaacctactcccagatcctaa

SEQ ID NO: 9 - DNA, 1482 bp, unidentified
  source 1..1482: mol_type = other DNA; note = TOT homologous gene; note (original language) = TOT同源基因
atggatacagttagagaattgaatggaggatcaggttcccctggtattcccctcagtctgatcaccgccgctgtgggtgccataataattctgtcactactgctcctccgccgttctaaacggggcaactcatctcatcctcctgggaattcagggcttccattcattggggagacattatcattcaccaaggcttttaaatcgaacacgctggaccaattttttgaggagagggtgaagaaattcgggcaagtctttaagctttccgtaatcgggcctcccacagtggcaatgtgcggccctgagggaaaccggtttgttttcgccaacgaggagaagcttgtccacttgtcgtggtctggtcgatatgcgaaaatcctgggtggagattccgtttccatgaagaggggagatgatcatcgcagagtacgtgccgcattcgcagggtttttgagccctgcatcactgcctgtttacataagtaaaatgagtgcacagatccaagatcatatcaacgaaaaatggaaagaaaaagttgtaattgctgtagttcctctggtaaaggagctcgtcttcaacgtttcctacaacttgtttttcagcataaatgatagcgaggaactgcatcgattgcataagattttcgaaactattgtggagggacatgtttccatgccgatagaccttcccggattcacctttcatagagcacttcagggaagggcgaagctcaagaaagttttctcttctttaatagaaaggagaagaagcgatctgagctccggattggcatctgctaatcaggatctcatctctgttttactcacctacaaagatgatagggggtatacaatgacccacgacgagctcctcgacaactttctttcccttcttgaatcctcctatgattccgtcaattcaccaatggcctgcatttttaagcttttgtatgacaatccagaatgctatgaaaaagtagttcaagagcaattggggatactttctggtaagaaggaaggacaagaaatctcgtggaaggatctgagatccatgaaatacacatggcaagtacttcaggaaacgctacgactgtatactcaagttgctggaatatttcgcaaagccatgactgacattcattatgatggtcacaccattcccaaagggtggcaacttctttgggcaacccaaactacacatctgaacgacaaatatttcagtgagccggaaaagttcatgccttccagattcgatgaagaaggaaacaatttgattccttactcattcgtaccatttggaggagggcggcggatgtgtccaggttgggaattcggaaagatggagatcttactctttgtccatcactttgttaaaacgttcagtggctttaccccaatcgatccggacgaaaaaattactgggaatccatttcctcatctccctgccaatggattttcaataaaacctactcccagatcctaa

SEQ ID NO: 10 - DNA, 1524 bp, unidentified
  source 1..1524: mol_type = other DNA; note = TOT homologous gene; note (original language) = TOT同源基因
atggttcatgtgttgcaggtagtgaaaatggatagagttagtgaaatatttaatggaagttcaggttctccagctggtattccccacagtgtgatcacagccggtgtgggtgccataataataattcttctgtcactagtgctcctccgccgttctagtaaacggggcgactcctctcatcctcctgggaattcaggccttccattcattggggagacattatcattcaccaaggcttttaaatcgaacacgctggccgaattttttgaggagagggtgaagaaattcgggaatgtatttaagatttcaataatcgggcctcccacagtggtaatgtgcggcaatgagggaaaccggtttattttcgccaacgaggagaagctgatgcacctgtcgtggtccggtcggtatgcgaaaatccttggtggggaatccgtttccatgaagaggggagatgatcatcgcagtgtacgtgccgcattcgcagggtttttgagcccttcggcgctgcctctttacgtagctaaaatgagtgcgcagatccaaaatcatatcaacgagaaatggaaaggaagagatgtaattgctgtagttcctttggtaaaagagctggtcttcaacgtttcctccaacttgtttttcagcatgaatgatagcgaggaattgcatctattgcatcaaattttcgaaactattgtagatggacatgtttccatgccgatagaccttcccggattcacctttcataaagcacttcagggaagggcgaagctcaagaaagtttactcttctttaatagaaaggagaagaagcgatctgagctccggattggcatctgctaatcaggatctcatctctgttttactcacctacaaagatgatagggggtatacaatgacccacgacgagctcctcgacaattttctttcccttattgaatcctcctatgattccatcaattcaccaatggcctgcatttttaagcttttgtatgccaatccagaatgctatgaaaaagtagttcaagagcaattggggatactttctggtaagaaggaaggagaagaaatctcatggaaggatctgagatccatgaaatacacatggcaagcaattcaggaaacgctacgaatttatactcaagttgcaggaatatttcgcaaagccatgactgacattcattatgatggtcacaccattcccaaagggtggcaacttctttgggcaacccaaactacacatctgaacgacaaatatttcagtgagcctgaaaaattcatgccttctagattcgatgaagaaggaaacaatgtgattccttactcattcgtaccatttggaggagggcggcggatgtgtccaggttgggaattcggaaagatggagatcttactctttgtccatcactttgttaaaacgttcagtggctttaccccaattgatccgaacgaaaaaattactgggaatccttttcctcatctccctgccaatggatttctaataaaacctattctcagatcctaa

SEQ ID NO: 11 - DNA, 1482 bp, unidentified
  source 1..1482: mol_type = other DNA; note = TOT homologous gene; note (original language) = TOT同源基因
atggatacagttagagaattgaatggaggatcaggttcccctggtattcccctcagtctgatcaccgccgctgtgggtgccataataattctgtcactactgctcctccgccgttctaaacggggcaactcatctcatcctcctgggaattcagggcttccattcattggggagacattatcattcaccaaggcttttaaatcgaacacgctggaccaatttttcgaggagagggtgaagaaattcgggcaagtctttaagctttccgtaatcgggcctcccacagtggcaatgtgcggccctgagggaaaccggtttgttttcgccaacgaggagaagcttgtccacttgtcgtggtctggtcgatatgcgaaaatcctgggtggagattccgtttccatgaagaggggagatgatcatcgcagtgtacgtgccgcattcgcagggtttttgagccctgcatcgctgcctgtttacataagtaaaatgagtgcacagatccaagatcatatcaacgaaaaatggaaaggaaaagatgtaattgctgtagttcctctggtaaaggagctcgtcttcaacgtttcctacaacttgtttttcagcttaaatgatagcgaggaactgcatcgattgcataagattttcgaaactattgtggagggacatgtttccatgccgatagaccttcccggattcacctttcatagagcacttcagggaagggcgaagctcaagaaagttttctcttctttaatagaaaggagaagaagcgatcttagctccggattggcatctgctaatcaggatctcatttctgttttactcacctacaaagatgatagggggtatacaatgacccacgacgagctcctcgacaactttctttcccttcttgaagcctcctatgattccgtcaattcaccaatggcctgcatttttaagcttttgtatgacaatccagaatgctatgaaaaagtagttcaagagcaattggggatactttctggtaagaaggaaggacaagaaatctcgtggaaggatctgagatccatgaaatacacatggcaagtacttcaggaaacgctacgactgtatactcaagttgctggaatatttcgcaaagccatgactgacattcattatgatggtcacaccattcccaaagggtggcaacttctttgggcaacccaaactacacatctgaacgacaaatatttcagtgagccggaaaagttcatgccttccagattcgatgaagaaggaaacaatttgattccttattcattcgtaccatttggaggagggcggcggatgtgtccaggttgggaattcggaaagatggagatcttactctttgtccatcactttgttaaaacgttcagtggctttaccccaatcgatccggacgaaaaaattactgggaatccatttcctcatctccctgccaatggattttcaataaaacctactcccagatcctaa

SEQ ID NO: 12 - DNA, 1497 bp, unidentified
  source 1..1497: mol_type = other DNA; note = TOT homologous gene; note (original language) = TOT同源基因
atggatagagttagagaaatatttaatggaagttcaggttctccagctggtattccccacagtgtgatcacagccggtgtgggtgccataataataattcttctgtcactactgctcctccgccgttctagtaaacggggcgactcctctcatcctcctgggaattcaggccttccattcattggggagacattatcattcaccaaggcttttaaatcgaacacgctggccgaattttttgaggagagggtgaagaaattcgggaatgtatttaagatttcaataatcgggcctcccacagtggtaatgtgcggcaatgagggaaaccggtttattttcgccaacgaggagaagctgatgcacctgtcgtggtccggtcgatatgcgaaaatccttggtggggaatccgtttccatgaagaggggagatgatcatcgcagtgtacgtgccgcattcgcagggtttttgagctctgcatcgctgcctgtttacataagtaaaatgagtgcacagatccaagatcatatcaacgaaaaatggaaaggaaaagatgtaattgctgtagttcctctggtaaaggagctcgtcttcaacgtttcctacaacttgtttttcagcataaatgatagcgaggaactgcatcgattgcataagattttcgaaactattgtggagggacatctttccatgccgatagaccttcccggattcacctttcatagagcacttcagggaagggcgaagctcaagaaagttttctcttctttaatagaaaggagaagaagcgatctgagctccggattggcatctgctaatcaggatctcatttctgttttactcacctacaaagatgatagggggtatacaatgacccacgacgagctcctcgacaactttctttcccttcttgaaggctcctatgattccatcaattcaccaatggcctgcatttttaagcttttgtatgacaatccagaatgctatgaaaaagtagttcaagagcaattggggatactttctggtaagaaggaaggacaagaaatctcgtggaaggatctgagatccatgaaatacacatggcaagtacttcaggaaacgctacgactgtatactcaagttgctggaatatttcgcaaagccatgactgacattcattatgatggtcacaccattcccaaagggtggcaacttctttgggcaaaccaaactacacatctgaacgacaaatatttcagtgagcctgaaaaattcatgccttccagattcgatgaagaaggaaacaatatgattccttactcattcgtaccatttggaggagggcggcggatgtgtccaggttgggaattcggaaagatggagatcttactctttgtccatcactttgttaaaacgttcagtggctttaccccaattgatccgaacgaaaaaattactgggaatccttttcctcatctccctgccaatggatttctaataaaacctattctcagatcctaa

SEQ ID NO: 13 - DNA, 1497 bp, unidentified
  source 1..1497: mol_type = other DNA; note = TOT homologous gene; note (original language) = TOT同源基因
atggatagagttagtgaaatatttaatggaagttcaggttctccagctggtattccccacagtgtgatcacagccggtgtgggtgccataataataattcttctgtcactagtgctcctccgccgttctagtaaacggggcgactcctctcatcctcctgggaattcaggccttccattcattggggagacattatcattcaccaaggcttttaaatcgaacacgctggccgaattttttgaggagagggtgaagaaattcgggaatgtatttaagatttcaataatcgggcctcccacagtggtaatgtgcggcaatgagggaaaccggtttattttcgccaacgaggagaagctgatgcacctgtcgtggtccggtcggtatgcgaaaatccttggtggggaatccgtttccatgaagaggggagatgatcatcgcagtgtacgtgccgcattcgcagggtttttgagcccttcggcgctgcctctttacgtagctaaaatgagtgcgcagatccaaaatcatatcaacgagaaatggaaaggaagagatgtaattgctgtagttcctttggtaaaagagctggtcttcaacgtttcctccaacttgtttttcagcatgaatgatagcgaggaattgcatctattgcatcaaattttcgaaactattgtagatggacatgtttccatgccgatagaccttcccggattcacctttcataaagcacttcagggaagggcgaagctcaagaaagtttactcttctttaatagaaaggagaagaagcgatctgagctccggattggcatctgctaatcaggatctcatctctgttttactcacctacaaagatgatagggggtatacaatgacccacgacgagctcctcgacaattttctttcccttattgaatcctcctatgattccatcaattcaccaatggcctgcatttttaagcttttgtatgccaatccagaatgctatgaaaaagtagttcaagagcaattggggatactttctggtaagaaggaaggagaagaaatctcatggaaggatctgagatccatgaaatacacatggcaagcaattcaggaaacgctacgaatttatactcaagttgcaggaatatttcgcaaagccatgactgacattcattatgatggtcacaccattcccaaagggtggcaacttctttgggcaacccaaactacacatctgaacgacaaatatttcagtgagcctgaaaaattcatgccttctagattcgatgaagaaggaaacaatgtgattccttactcattcgtaccatttggaggagggcggcggatgtgtccaggttgggaattcggaaagatggagatcttactctttgtccatcactttgttaaaacgttcagtggctttaccccaattgatccgaacgaaaaaattactgggaatccttttcctcatctccctgccaatggatttctaataaaacctattctcagatcctaa

SEQ ID NO: 14 - DNA, 1524 bp, unidentified
  source 1..1524: mol_type = other DNA; note = TOT homologous gene; note (original language) = TOT同源基因
atggttcatgtgttgcaggtagtgaaaatggatagagttagagaaatatttaatggaagttcaggttctccagctggtattccccacagtgtgatcacagccggtgtgggtgccataataataattcttctgtcactactgctcctccgccgttctagtaaacggggcgactcctctcatcctcctgggaattcaggccttccattcattggggagacattatcattcaccaaggcttttaaatcgaacacgctggccgaattttttgaggagagggtgaagaaattcgggaatgtatttaagatttcaataatcgggcctcccacagtggtaatgtgcggcaatgagggaaaccggtttattttcgccaacgaggagaagctgatgcacctgtcgtggtccggtcgatatgcgaaaatccttggtggggaatccgtttccatgaagaggggagatgatcatcgcagtgtacgtgccgcattcgcagggtttttgagccctgcatcgctgcctatttacataagtaaaatgagtgcacagatccaagatcatatcaacaaaaaatggaaaggaaaagatgtaattgctgtagttcctctggtaaaggagctcgtcttcaacgtttcctacaacttgtttttcagcataaatgatagcgaggaacttcatcgattgcataagattttcgaaactattgtggagggacatgtttccatgccgatagaccttcccggattcacctttcatagagcacttcagggaagggcgaagctcaagaaagtttactcttctttaatagaaaggagaagaagcgatctgagctccggattggcatctgctaatcaggatcttatctctgttttactcacctacaaagatgatagggggtatagaatgacccacgacgagctcctcgacaactttctttcccttcttgaatcctcctatgattccgtcaattcaccaatggcctgcattttaaagcttttgtatgccaatccagaatgctatgaaaaagtagttcaagagcaattggggatactttctggtaagaaggaaggagaagaaatctcatggaaggatctgagatccatgaaatacacatggcaagtacttcaggaaacgctacgactgtatactcaagttgctggaatatttcgcaaagccatgactgacattcattatgatggtcacaccattcccaaagggtggcaacttctttgggcaacccaaactacacatctgaacgacaaatatttcagtgagcctgaaaaattcatgccttccagattcgatgaagaaggaaacaatgtgattccttactcattcgtaccatttggaggagggcggcggatgtgtccaggttgggaattcggaaagatggagatcttactctttgtccatcactttgttaaaacgttcagtggctttaccccaattgatccgaacgaaaaaattactgggaatccttttcctcatctccctgccaatggatttctaataaaacctattctcagatcctaa

SEQ ID NO: 15 - DNA, 1524 bp, unidentified
  source 1..1524: mol_type = other DNA; note = TOT homologous gene; note (original language) = TOT同源基因
atggttcatgtgttgcaggtagtgaaaatggatagagttagagaaatatttaatggaagttcaggttctccagctggtattccccacagtgtgatcacagccggtgtgggtgccataataataattcttctgtcactactgctcctccgccgttctagtaaacggggcgactcctctcatcctcctgggaattcaggccttccattcattggggagacattatcattcaccaaggcttttaaatcgaacacgctggccgaattttttgaggagagggtgaagaaattcgggaatgtatttaagatttcaataatcgggcctcccacagtggtaatgtgcggcaatgagggaaaccggtttattttcgccaacgaggagaagctgatgcacctgtcgtggtccggtcgatatgcgaaaatccttggtggggaatccgtttccatgaagaggggagatgatcatcgcagtgtacgtgccgcattcgcagggtttttgagcccttcggcgctgcctctttacgtagctaaaatgagtgcgcagatccaaaatcatatcaacgagaaatggaaaggaagagatgtaattgccgtagttcctttggtaaaagagctggtcttcaacgtttcctccaacttgtttttcagcatgaatgatagcgaggaactgcatcgattgcatcaaattttcgaaactattgtagatggacatgtttccatgcccatagaccttcccggattcacctttcataaagcacttcagggaagggcgaagctcaagaaagtttactcttctttaatagaaaggagaagaagcgatctgagctccggattggcatctgctaatcaggatcttatctctgttttactcacctacaaagatgatagggggtatagaatgacccacgacgagctcctcgacaactttctttcccttcttgaatcctcctatgattccgtcaattcaccaatggcctgcattttaaagcttttgtatgccaatccagaatgctatgaaaaagtagttcaagagcaattggggatactttctggtaagaaggaaggagaagaaatctcatggaaggatctgagatccatgaaatacacatggcaagtacttcaggaaacgctacgactgtatactcaagttgctggaatatttcgcaaagccatgactgacattcattatgatggtcacaccattcccaaagggtggcaacttctttgggcaacccaaactacacatctgaacgacaaatatttcagtgagcctgaaaaattcatgccttccagattcgatgaagaaggaaacaatgtgattccttactcattcgtaccatttggaggagggcggcggatgtgtccaggttgggaattcggaaagatggagatcttactctttgtccatcactttgttaaaacgttcagtggctttaccccaattgatccgaacgaaaaaattactgggaatccttttcctcatctccctgccaatggatttctaataaaacctattctcagatcctaa

SEQ ID NO: 16 - DNA, 1497 bp, unidentified
  source 1..1497: mol_type = other DNA; note = TOT homologous gene; note (original language) = TOT同源基因
atggatagagttagagaaatatttaatggaagttcaggttctccagctggtattccccacagtgtgatcacagccggtgtgggtgccataataataattcttctgtcactactgctcctccgccgttctagtaaacggggcgactcctctcatcctcctgggaattcaggccttccattcattggggagacattatcattcaccaaggcttttaaatcgaacacgctggccgaattttttgaggagagggtgaagaaattcgggaatgtatttaagatttcaataatcgggcctcccacagtggtaatgtgcggcaatgagggaaaccggtttattttcgccaacgaggagaagctgatgcacctgtcgtggtccggtcgatatgcgaaaatccttggtggggaatccgtttccatgaagaggggagatgatcatcgcagtgtacgtgccgcattcgcagggtttttgagccctgcatcgctgcctatttacataagtaaaatgagtgcacagatccaagatcatatcaacaaaaaatggaaaggaaaagatgtaattgctgtagttcctctggtaaaggagctcgtcttcaacgtttcctacaacttgtttttcagcataaatgatagcgaggaacttcatcgattgcataagattttcgaaactattgtggagggacatgtttccatgccgatagaccttcccggattcacctttcatagagcacttcagggaagggcgaagctcaagaaagtttactcttctttaatagaaaggagaagaagcgatctgagctccggattggcatctgctaatcaggatcttatctctgttttactcacctacaaagatgatagggggtatagaatgacccacgacgagctcctcgacaactttctttcccttcttgaatcctcctatgattccgtcaattcaccaatggcctgcattttaaagcttttgtatgccaatccagaatgctatgaaaaagtagttcaagagcaattggggatactttctggtaagaaggaaggagaagaaatctcatggaaggatctgagatccatgaaatacacatggcaagtacttcaggaaacgctacgactgtatactcaagttgctggaatatttcgcaaagccatgactgacattcattatgatggtcacaccattcccaaagggtggcaacttctttgggcaacccaaactacacatctgaacgacaaatatttcagtgagcctgaaaaattcatgccttccagattcgatgaagaaggaaacaatgtgattccttactcattcgtaccatttggaggagggcggcggatgtgtccaggttgggaattcggaaagatggagatcttactctttgtccatcactttgttaaaacgttcagtggctttaccccaattgatccgaacgaaaaaattactgggaatccttttcctcatctccctgccaatggatttctaataaaacctattctcagatcctaa

SEQ ID NO: 17 - DNA, 1497 bp, unidentified
  source 1..1497: mol_type = other DNA; note = TOT homologous gene; note (original language) = TOT同源基因
atggatagagttagagaaatatttaatggaagttcaggttctccagctggtattccccacagtgtgatcacagccggtgtgggtgccataataataattcttctgtcactactgctcctccgccgttctagtaaacggggcgactcctctcatcctcctgggaattcaggccttccattcattggggagacattatcattcaccaaggcttttaaatcgaacacgctggccgaattttttgaggagagggtgaagaaattcgggaatgtatttaagatttcaataatcgggcctcccacagtggtaatgtgcggcaatgagggaaaccggtttattttcgccaacgaggagaagctgatgcacctgtcgtggtccggtcgatatgcgaaaatccttggtggggaatccgtttccatgaagaggggagatgatcatcgcagtgtacgtgccgcattcgcagggtttttgagcccttcggcgctgcctctttacgtagctaaaatgagtgcgcagatccaaaatcatatcaacgagaaatggaaaggaagagatgtaattgccgtagttcctttggtaaaagagctggtcttcaacgtttcctccaacttgtttttcagcatgaatgatagcgaggaactgcatcgattgcatcaaattttcgaaactattgtagatggacatgtttccatgcccatagaccttcccggattcacctttcataaagcacttcagggaagggcgaagctcaagaaagtttactcttctttaatagaaaggagaagaagcgatctgagctccggattggcatctgctaatcaggatcttatctctgttttactcacctacaaagatgatagggggtatagaatgacccacgacgagctcctcgacaactttctttcccttcttgaatcctcctatgattccgtcaattcaccaatggcctgcattttaaagcttttgtatgccaatccagaatgctatgaaaaagtagttcaagagcaattggggatactttctggtaagaaggaaggagaagaaatctcatggaaggatctgagatccatgaaatacacatggcaagtacttcaggaaacgctacgactgtatactcaagttgctggaatatttcgcaaagccatgactgacattcattatgatggtcacaccattcccaaagggtggcaacttctttgggcaacccaaactacacatctgaacgacaaatatttcagtgagcctgaaaaattcatgccttccagattcgatgaagaaggaaacaatgtgattccttactcattcgtaccatttggaggagggcggcggatgtgtccaggttgggaattcggaaagatggagatcttactctttgtccatcactttgttaaaacgttcagtggctttaccccaattgatccgaacgaaaaaattactgggaatccttttcctcatctccctgccaatggatttctaataaaacctattctcagatcctaa

SEQ ID NO: 18 - DNA, 1524 bp, unidentified
  source 1..1524: mol_type = other DNA; note = TOT homologous gene; note (original language) = TOT同源基因
atggttcatgtgttgcaggtagtgaaaatggatagagtcagtgaaatatttaatggaagttcaggttctccagctggtattccccacagtgtgatcacagccggtgtgggtgccataataataattcttctgtcactactgctcctccgccgttctagtaaacggggcgactcctctcatcctcctgggaattcaggccttccattcattggggagacattatcattcaccaaggcttttaaatcgaacacgctggccgaattttttgaggagagggtgaagaaattcgggaatgtatttaagatttcaataatcgggcctcccacagtggtaatgtgcggcaatgagggaaaccggtttattttcgccaacgaggagaagctgatgcacctgtcgtggtccggtcgatatgcgaaaatccttggtggggaatccgtttccatgaagaggggagatgatcatcgcagtgtacgtgccgcattcgcagggtttttgagcccttcggcgctgcctctttacgtagctaaaatgagtgcgcagatccaaaatcatatcaacgagaaatggaaaggaagagatgtaattgccgtagttcctttggtaaaagagctggtcttcaacgtttcctccaacttgtttttcagcatgaatgatagcgaggaactgcatcgattgcatcaaattttcgaaactattgtagatggacatgtttccatgcccatagaccttcccggattcacctttcataaagcacttcagggaagggcgaagctcaagaaagtttactcttctttaatagaaaggagaagaagcgatctgagctccggattggcatctgctaatcaggatctcatctctgttttactcacctacaaagatgatagggggtatacaatgacccatgacgagctcctcgacaattttctttcccttattgaatcctcctatgattccatcaattcaccaatggcctgcatttttaagcttttgtatgccaatccagaatgctatgaaaaagtagttcaagagcaattggggatactttctggtaagaaggaaggagaagaaatctcatggaaggatctgagatccatgaaatacacatggcaagcaattcaggaaacgctacgaatttatactcaagttgcaggaatatttcgcaaagccatgactgacattcattatgatggtcacaccattcccaaagggtggcaacttctttgggcaacccaaactacacatctgaacgacaaatatttcagtgagcctgaaaaattcatgccttccagattcgatgaagaaggaaacaatgtgattccttactcattcgtaccatttggaggagggcggcggatgtgtccaggttgggaattcggaaagatggagatcttactctttgtccatcactttgttaaaacgttcagtggctttaccccaattgatccgaacgaaaaaattactgggaatccttttcctcatctccctgccaatggatttctaataaaacctattctcagatcctaa

SEQ ID NO: 19 - DNA, 1494 bp, unidentified
  source 1..1494: mol_type = other DNA; note = TOT homologous gene; note (original language) = TOT同源基因
atggatgtcttttatccgttaaaaagtgcagtaacaaaatttaacgaatgtttccctgctattcttttcattgtcctcagtgctgttgctggcattgttctgcccctgctgctgttcctacgttctaaacgccgttcctctgttggactacccccagggaaattaggttaccctttcattggcgagtcgttactgttcctgaaggctcttcgatcaaacacagttgagcaatttttggacgagagagtgaagaaattcgggaatgtcttcaagacgtcattaattgggcatccgacagtagttctctgcgggcctgcgggaaaccggctaatcctggcgaacgaggagaagctggtgcagatgtcgtggcccaaatcctctatgaaactcatgggggaaaagtctatcaccgccaaaaggggcgaaggccatatgatcatccgctccgcactgcaaggctttttcagccctggtgctctgcagaaatacataggccaaatgagtaaaacaatagaaaatcatattaatgagaaatggaagggcaacgaccaagtgagtgtagttgctttggtaggagatctcgtcttcgatatatcggcctgtttgttcttcaatataaatgagaagcatgaacgggaacgactgtttgagcttttggagattatagctgtcggagttttggctgttccggtggatcttcccggatttgcttaccgtcgggcacttcaagcacggtcgaagcttaatgcaattctctccggtttgatagaaaagagaaaaatggatctgagctcaggattagcgagtagcaatcaggatcttctttctgtgtttctcaccttcaaagatgacagaggaaatccactgagcgatgaggaaatcctcgacaacttttccgggctgcttcatggatcctatgacaccactgtttcagcaatggcctgcgtttttaagcttttgtcttccaatcccgaatgctatgaaaaagtagttcaagagcaattggggatactttctggtaagaaggaaggacaagaaatctcgtggaaggatctgagatccatgaaatacacatggcaagtacttcaggaaacgctacgactgtatactcaagttgctggaatatttcgcaaagccatgactgacattcattatgatggtcacaccattcccaaagggtggcaacttctttgggcaacccaaactacacatctgaacgacaaatatttcagtgagccggaaaaattcatgccttccagattcgatgaagaaggaaacaatgtgattccttactcattcgtaccatttggaggagggcggcggatgtgtccaggttgggaattcggaaagatggagatcttactcttcgtccatcactttgttaaagcgttcagtggctttaccccaatcgatccggacgaaaaaattactgggaatccttttcctcatctccctgccaatggatttctaataaaacctattctcagatcctaa

SEQ ID NO: 20 - DNA, 1497 bp, unidentified
  source 1..1497: mol_type = other DNA; note = TOT homologous gene; note (original language) = TOT同源基因
atggatagagtcagtgaaatatttaatggaagttcaggttctccagctggtattccccacagtgtgatcacagccggtgtgggtgccataataataattcttctgtcactactgctcctccgccgttctagtaaacggggcgactcctctcatcctcctgggaattcaggccttccattcattggggagacattatcattcaccaaggcttttaaatcgaacacgctggccgaattttttgaggagagggtgaagaaattcgggaatgtatttaagatttcaataatcgggcctcccacagtggtaatgtgcggcaatgagggaaaccggtttattttcgccaacgaggagaagctgatgcacctgtcgtggtccggtcgatatgcgaaaatccttggtggggaatccgtttccatgaagaggggagatgatcatcgcagtgtacgtgccgcattcgcagggtttttgagcccttcggcgctgcctctttacgtagctaaaatgagtgcgcagatccaaaatcatatcaacgagaaatggaaaggaagagatgtaattgccgtagttcctttggtaaaagagctggtcttcaacgtttcctccaacttgtttttcagcatgaatgatagcgaggaactgcatcgattgcatcaaattttcgaaactattgtagatggacatgtttccatgcccatagaccttcccggattcacctttcataaagcacttcagggaagggcgaagctcaagaaagtttactcttctttaatagaaaggagaagaagcgatctgagctccggattggcatctgctaatcaggatctcatctctgttttactcacctacaaagatgatagggggtatacaatgacccatgacgagctcctcgacaattttctttcccttattgaatcctcctatgattccatcaattcaccaatggcctgcatttttaagcttttgtatgccaatccagaatgctatgaaaaagtagttcaagagcaattggggatactttctggtaagaaggaaggagaagaaatctcatggaaggatctgagatccatgaaatacacatggcaagcaattcaggaaacgctacgaatttatactcaagttgcaggaatatttcgcaaagccatgactgacattcattatgatggtcacaccattcccaaagggtggcaacttctttgggcaacccaaactacacatctgaacgacaaatatttcagtgagcctgaaaaattcatgccttccagattcgatgaagaaggaaacaatgtgattccttactcattcgtaccatttggaggagggcggcggatgtgtccaggttgggaattcggaaagatggagatcttactctttgtccatcactttgttaaaacgttcagtggctttaccccaattgatccgaacgaaaaaattactgggaatccttttcctcatctccctgccaatggatttctaataaaacctattctcagatcctaa

SEQ ID NO: 21 - DNA, 1524 bp, unidentified
  source 1..1524: mol_type = other DNA; note = TOT homologous gene; note (original language) = TOT同源基因
atggttcatgtgttgcaggtagtgaaaatggatagagttaatgaaatatttaatggaagttcaggttctccagctggtattccccacagtgtgatcacagccggtgtgggtgccataataataattcttctgtcactactgctcctccgccgttctagtaaacggggcgactccgctcatcctcctgggaattcaggccttccattcattggggagacattatcattcaccaaggcttttaaatcgaacacgctggccgaattttttgaggagagggtgaagaaattcgggaatgtatttaagatttcaataatcgggcctcccacagtggtaatgtgcggcaatgagggaaaccggtttattttcgccaacgaggagaagctgatgcacctgtcgtggtccggtcgatatgcgaaaatccttggtggggaatccgtttccatgaagaggggagatgatcatcgcagtgtacgtgccgcattcgcagggtttttgagctctgcatcgctgcctgtttacataagtaaaatgagtgcacagatccaagatcatatcaacgaaaaatggaaaggaaaagatgtaattgctgtagttcctctggtaaaggagctcgtcttcaacgtttcctacaacttgtttttcagcataaatgatagcgaggaactgcatcgattgcataagattttcgaaactattgtggagggacatgtttccatgccgatagaccttcccggattcacctttcatagagcacttcagggaagggagaagctcaagaaagttttctcttctttaatagaaaggagaagaagcgatcttagctccggattggcatctgctaatcaggatctcatttctgttttactcacctacaaagatgatagggggtatacaatgacccacgacgagctcctcgacaactttctttcccttcttgaatcctcctatgattccgtcaattcaccaatggcctgcatttttaagcttttgtatgacaatccagaatgctatgaaaaagtagttcaagagcaattggggatactttctggtaagaaggaaggacaagaaatctcgtggaaggatctgagatccatgaaatacacatggcaagtacttcaggaaacgctacgactgtatactcaagttgctggaatatttcgcaaagccatgactgacattcattatgatggtcacaccattcccaaagggtggcaacttctttgggcaacccaaactacacatctgaacgacaaatatttcagtgagccggaaaagttcatgccttccagattcggtgaagaaggaaacaatttgattccttactcattcgtaccatttggaggagggcggcggatgtgtccaggttgggaattcggaaagatggagatcttactctttgtccatcactttgttaaaacgttcagtggctttaccccaatcgatccggacgaaaaaattactgggaatccatttcctcatctccctgccaatggattttcaataaaacctactcccagatcctaa

SEQ ID NO: 22 - DNA, 1497 bp, unidentified
  source 1..1497: mol_type = other DNA; note = TOT homologous gene; note (original language) = TOT同源基因
atggatagagttaatgaaatatttaatggaagttcaggttctccagctggtattccccacagtgtgatcacagccggtgtgggtgccataataataattcttctgtcactactgctcctccgccgttctagtaaacggggcgactccgctcatcctcctgggaattcaggccttccattcattggggagacattatcattcaccaaggcttttaaatcgaacacgctggccgaattttttgaggagagggtgaagaaattcgggaatgtatttaagatttcaataatcgggcctcccacagtggtaatgtgcggcaatgagggaaaccggtttattttcgccaacgaggagaagctgatgcacctgtcgtggtccggtcgatatgcgaaaatccttggtggggaatccgtttccatgaagaggggagatgatcatcgcagtgtacgtgccgcattcgcagggtttttgagctctgcatcgctgcctgtttacataagtaaaatgagtgcacagatccaagatcatatcaacgaaaaatggaaaggaaaagatgtaattgctgtagttcctctggtaaaggagctcgtcttcaacgtttcctacaacttgtttttcagcataaatgatagcgaggaactgcatcgattgcataagattttcgaaactattgtggagggacatgtttccatgccgatagaccttcccggattcacctttcatagagcacttcagggaagggagaagctcaagaaagttttctcttctttaatagaaaggagaagaagcgatcttagctccggattggcatctgctaatcaggatctcatttctgttttactcacctacaaagatgatagggggtatacaatgacccacgacgagctcctcgacaactttctttcccttcttgaatcctcctatgattccgtcaattcaccaatggcctgcatttttaagcttttgtatgacaatccagaatgctatgaaaaagtagttcaagagcaattggggatactttctggtaagaaggaaggacaagaaatctcgtggaaggatctgagatccatgaaatacacatggcaagtacttcaggaaacgctacgactgtatactcaagttgctggaatatttcgcaaagccatgactgacattcattatgatggtcacaccattcccaaagggtggcaacttctttgggcaacccaaactacacatctgaacgacaaatatttcagtgagccggaaaagttcatgccttccagattcggtgaagaaggaaacaatttgattccttactcattcgtaccatttggaggagggcggcggatgtgtccaggttgggaattcggaaagatggagatcttactctttgtccatcactttgttaaaacgttcagtggctttaccccaatcgatccggacgaaaaaattactgggaatccatttcctcatctccctgccaatggattttcaataaaacctactcccagatcctaa

SEQ ID NO: 23 - DNA, 1524 bp, unidentified
  source 1..1524: mol_type = other DNA; note = TOT homologous gene; note (original language) = TOT同源基因
atggttcatgtgttgcaggtagtgaaaatggatagagttagtgaaatatttaatggaagttcaggttctccagctggtattccccacagtgtgatcacagccggtgtgggtgccataataataattcttctgtcactagtgctcctccgccgttctagtaaacggggcgactcctctcatcctcctgggaattcaggccttccattcattggggagacattatcattcaccaaggcttttaaatcgaacacgctggccgaattttttgaggagagggtgaagaaattcgggaatgtatttaagatttcaataatcgggcctcccacagtggtaatgtgcggcaatgagggaaaccggtttattttcgccaacgaggagaagctgatgcacctgtcgtggtccggtcgatatgcgaaaatccttggtggggaatccgtttccatgaagaggggagatgatcatcgcagtgtacgtgccgcattcgcagggtttttgagcccttcggcgctgcctctttacgtagctaaaatgagtgcgcagatccaaaatcatatcaacgagaaatggaaaggaagagatgtaattgctgtagttcctttggtaaaagagctggtcttcaacgtttcctccaacttgtttttcggcatgaatgatagcgaggaactgcatcgattgcatcaaattttcgaaactattgtagatggacatgtttccatgccgatagaccttcccggattcacctttcataaagcacttcagggaagggcgaagctcaagaaagtttactcttctttaatagaaaggagaagaagcgatctgagctccggattggcatctgctaatcaggatctcatctctgttttactcacctacaaagatgatagggggtatacaatgacccacgtcgagctcctcgacaattttctttcccttattgaatcctcctatgattccatcaattcaccaatggcctgcatttttaagcttttgtatgccaatccagaatgctatgaaaaagtagttcaagagcaattggggatactctctggtaagaagaaaggagaagaaatctcatggaaggatctgagatccatgaaatacacatggcaagcaattcaggaaacgctacgaatttatactcaagttgcaggaatatttcgcaaagccatgactgacattcattatgatggtcacaccattcccaaagggtggcaacttctttgggcaacccaaactacacatctgaacgacaaatatttcagtgagcctgaaaaattcatgccttccagattcgatgaagaaggaaacaatgtgattccttactcattcgtaccatttggaggagggcggcggatgtgtccaggttgggaattcggaaagatggagatcttactctttgtccatcactttgttaaaacgttcagtggctttaccccaattgatccgaacgaaaaaattactgggaatccttttcctcatctccctgccaatggatttctaataaaacctattctcagatcctaa

SEQ ID NO: 24 - DNA, 1533 bp, unidentified
  source 1..1533: mol_type = other DNA; note = TOT homologous gene; note (original language) = TOT同源基因
atggattccttgcatcgtgtaatcaagatctctgcaatatttaatggagacaccaaactacactggtcctcccctgctgttttttctgttgccttcactgctgttgccggcatacttcttctgttactgctcctccgttctaaacgccgccactcctctctgaatcagtacaatcttcctcgtggaaattcaggcctccctttcgttggggagacgatatcattcctgagggcctttcgaggaaacagaattcaacaattcttcgacgagagagcgaaaaaattcggaaatgtcttcaggatttcgataactgggcctcccacggcagtactgtgcggctcagagggaaaccgctttattctctccaacgaggagaagctggtgcgggttgacatgtccggagcattttccaaactggctggtcgggattccgtcatgatgagaacgggcgaggagcatcgcaccatacgagcagctatggcaggttttttggcccctacagcgctacccatttacgtgggtaaaatgagtgcacagatccaaaatcatatcgatgaaaaatggaaaggaaaagatgtggttactgtagtttctctcgtaaaagagctggtcttcggcgtttcagccagcatgttttacgatataaatgatggtgtcgaacagcatcgactgcacgagatttaccaaactatggttgcgggccatttttcttttccgctagattttcccggattttcttttcatagagcagttcagggaaggcagaagctcaagaaaattttctcttctttaatagaaaagaggagaagcgatctgcgctcgggattagcatctagcaatcaagatctactctccgttttgctcacctacaaaaatgaaaaagggaatggactcacgcagggtgagctcaccgacaactttattaccatgctcgaagcctcttatgacaaccccgtttcagccatttcctgtattctcaagttcttgtattcccatcccgaagtgtatgaaaaagtagttcaagagcaattgggcatactttcaaataaagaggagggagacgaaatctcatggaaggatgttaaagccatgaaatacacatggcaagctgtccaggaaacgttacgaatgatttctccagtgattggaatactgagaaaggccatgacagacattcattatgatggctacacaattccgaaaggatggcaactcctatggacaggctgcagtacacatctgaaagatgcatattttaatgaggcggacgaattcatgccttcaagattcgatgaggaaggaaagaatgtggttccttactcgtttgtgccatttggaggagggcgtcggatgtgtccaggatgggaattctctaaactggcgatactactgttcgtccatcactttgttaaaacattcagtagttacaccccacttgatcccgacgaaaaaattcttgggaatccattccctctcctccctgtcaatggactttccattaaacttactgccagatctgaaattaagaattaa

SEQ ID NO: 25 - protein, 507 aa, unidentified
  source 1..507: note = TOT reference protein; note (original language) = TOT参考蛋白
MVHVLQVVKMDRVREIFNGSSGSPAGIPHSVITAGVGAIIIILLSLLLLRRSSKRGDSSHPPGNSGLPFIGETLSFTKAFKSNTLAEFFEERVKKFGNVFKISIIGPPTVVMCGNEGNRFIFANEEKLVHLSWSGRYAKILGGDSVSMKRGDDHRSVRAAFAGFLSPASLPIYISKMSAQIQDHINQKWKGKDVIAVVPLVKELVFNVSYNLFFSINDSEELHRLHKIFETIVEGHVSMPIDLPGFTFHRALQGRAKLKKVFSSLIERRRSDLSSGLASANQDLISVLLTYKDDRGYTMTHDELLDNFLSLLESSYDSVNSPMACIFKLLYANPECYEKVVQEQLGILSGKKEGQEISWKDLRSMKYTWQVLQETLRLYTQVAGIFRKAMTVIHYDGHTIPKGWQLLWATQTTHLNDKYFSEPEKFMPSRFDEEGNNVIPYSFVPFGGGRRMCPGWEFGKMEILLFVHHFVKAFSGFTPIDPDEKITGNPFPHLPANGFSIKPTPRS

SEQ ID NO: 26 - protein, 507 aa, unidentified
  source 1..507: note = TOT homologous protein; note (original language) = TOT同源蛋白
MVHVLQVVKMDRVSEIFNGSSGSPAGIPHSVITAGVGAIIIILLSLVLLRRSSKRGDSSHPPGNSGLPFIGETLSFTKAFKSNTLAEFFEERVKKFGNVFKISIIGPPTVVMCGNEGNRFIFANEEKLMHLSWSGRYAKILGGESVSMKRGDDHRSVRAAFAGFLSPSALPLYVAKMSAQIQNHINEKWKGRDVIAVVPLVKELVFNVSSNLFFSMNDSEELHRLHQIFETIVDGHVSMPIDLPGFTFHKALQGRAKLKKVYSSLIERRRSDLSSGLASANQDLISVLLTYKDDRGYTMTHDELLDNFLSLIESSYDSINSPMACIFKLLYANPECYEKVVQEQLGILSGKKEGEEISWKDLRSMKYTWQAIQETLRIYTQVAGIFRKAMTDIHYDGHTIPKGWQLLWATQTTHLNDKYFSEPEKFMPSRFDEEGNNVIPYSFVPFGGGRRMCPGWEFGKMEILLFVHHFVKTFSGFTPIDPNEKITGNPFPHLPANGFLIKPILRS

SEQ ID NO: 27 - protein, 507 aa, unidentified
  source 1..507: note = TOT homologous protein; note (original language) = TOT同源蛋白
MVHVLHVVKMDRVREIFNGSSGSPAGIPHSVITAGVGAIIIILLSLLLLRRSSKRGDSSHPPGNSGLPFIGETLSFTKAFKSNTLAEFFEERVKKFGNVFKISIIGPPTVVMCGNEGNRFIFANEEKLMHLSWSGRYAKILGGESVSMKRGDDHRSVRAAFAGFLSSASLPVYISKMSAQIQDHINEKWKGKDVIAVVPLVKELVFNVSYNLFFSINDSEELHRLHKIFETIVEGHLSMPIDLPGFTFHRALQGRAKLKKVFSSLIERRRSDLSSGLASANQDLISVLLTYKDDRGYTMTHDELLDNFLSLLEGSYDSINSPMACIFKLLYDNPECYEKVVQEQLGILSGKKEGQEISWKDLRSMKYTWQVLQETLRLYTQVAGIFRKAMTDIHYDGHTIPKGWQLLWANQTTHLNDKYFSEPEKFMPSRFDEEGNNMIPYSFVPFGGGRRMCPGWEFGKMEILLFVHHFVKTFSGFTPIDPNEKITGNPFPHLPANGFLIKPILRS

SEQ ID NO: 28 - protein, 507 aa, unidentified
  source 1..507: note = TOT homologous protein; note (original language) = TOT同源蛋白
MVHVLQVVKMDRVSEIFNGSSGSPAGIPHSVITAGVGAIIIILLSLVLLRRSSKRGDSSHPPGNSGLPFIGETLSFTKAFKSNTLAEFFEERVKKFGNVFKISIIGPPTVVMCGNEGNRFIFANEEKLMHLSWSGRYAKILGGESVSMKRGDDHRSVRAAFAGFLSPSALPLYVAKMSAQIQNHINEKWKGRDVIAVVPLVKELVFNVSSNLFFSMNDSEELHRLHQIFETIVDGHVSMPIDLPGFTFHKALQGRAKLKKVYSSLIERRRSDLSSGLASANQDLISVLLTYKDDRGYTMTHDELLDNFLSLIESSYDSVNSPMACIFKLLYANPECYEKVVQEQLGILSGKKEGQEISWKDLRSMKYTWQVLQETLRLYTQVAGIFRKAMTVIHYDGHTIPKGWQLLWATQTTHLNDKYFSEPQKFMPSRFDEEGNNVIPYSFVPFGGGRRMCPGWEFGKMEILLFVHHFVKAFSGFTPIDPDEKITGNPFPHLPANGFLIKPILRS

SEQ ID NO: 29 - protein, 493 aa, unidentified
  source 1..493: note = TOT homologous protein; note (original language) = TOT同源蛋白
MDTVRELNGGSGSSGIPLSLITAAVGAIIILSLLLLRRSKRGNSSHPPGNSGLPFIGETLSFTKAFKSNTLDQFFEERVKKFGQVFKLSVIGPPTVAMCGPEGNRFVFANEEKLVHLSWSGRYAKILGGDSVSMKRGDDHRSVRAAFAGFLSPASLPVYISKMSAQIQDHINEKWKGKDVIAVVPLVKELVFNVSYNLFFSINDSEELHRLHKIFETIVEGHVSMPIDLPGFTFHRALQGRAKLKKVFSSLIERRRSDLSSGLASANQDLISVLLTYKDDRGYTMTHDELLDNFLSLLEASYDSVNSPMACIFKLLYANPECYEKVVQEQLGILSGKKEGQEISWKDLRSMKYTWQVLQETLRLYTQVAGIFRKAMTDIHYNGHTIPKGWQLLWATQTTHLNDKYFSEPEKFMPSRFDEEGNNVIPYSFVPFGGGRRMCPGWEFGKMEILLFVHHFVKAFSGFTPIDPDEKITGNPFPHLPANGFSIKPTPRS

SEQ ID NO: 30 - protein, 507 aa, unidentified
  source 1..507: note = TOT homologous protein; note (original language) = TOT同源蛋白
MVHVLQVVKMDRVSEIFNGSSGSPAGIPHSVITAGVGAIIIILLSLVLLRRSSKRGDSSHPPGNSGLPFIGETLSFTKAFKSNTLAEFFEERVKKFGNVFKISIIGPPTVVMCGNEGNRFIFANEEKLMHLSWSGRYAKILGGESVSMKRGDDHRSVRAAFAGFLSPSALPLYVAKMSAQIQNHINEKWKGRDVIAVVPLVKELVFNVSSNLFFGMNDSEELHRLHQIFETIVDGHVSMPIDLPGFTFHKALQGRAKLKKVYSSLIERRRSDLSSGLASANQDLISVLLTYKDDRGYTMTHVELLDNFLSLIESSYDSINSPMACIFKLLYANPECYEKVVQEQLGILSGKKEGEEISWKDLRSMKYTWQAIQETLRIYTQVAGIFRKAMTDIHYDGHTIPKGWQLLWATQTTHLNDKYFSEPEKFMPSRFDEEGNNVIPYSFVPFGGGRRMCPGWEFGKMEILLFVHHFVKTFSGFTPIDPNEKITGNPFPHLPANGFLIKPILRS

SEQ ID NO: 31 - protein, 507 aa, unidentified
  source 1..507: note = TOT homologous protein; note (original language) = TOT同源蛋白
MVHVLQVVKMYRVSEIFNGSSGSPAGIPHSVITAGVGAIIIILLSLVLLRRSSKRGDSSHPPGNSGLPFIGETLSFTKAFKSNTLAEFFEERVKKFGNVFKISIIGPPTVVMCGNEGNRFIFANEEKLMHLSWSGRYAKILGGESVSMKRGDDHRSVRAAFAGFLSPSALPLYVAKMSAQIQNHINEKWKGRDVIAVVPLVKELVFNVSSNLFFSMNDSEELHRLHQIFETIVDGHVSMPIDLPGFTFHKALQGRAKLKKVYSSLIERRRSDLSSGLASANQDLISVLLTYKDDRGYTMTHDELLDNFLSLIESSYDSINSPMACIFKLLYANPECYEKVVQEQLGILSGKKEGEEISWKDLRSMKYTWQAIQETLRIYTQVAGIFRKAMTDIHYDGHTIPKGWQLLWATQTTHLNDKYFSEPEKFMPSRFDEEGNNVIPYSFVPFGGGRRMCPGWEFGKMEILLFVHHFVKTFSGFTPIDPNEKITGNPFPHLPANGFLIKPILRS

SEQ ID NO: 32 - protein, 493 aa, unidentified
  source 1..493: note = TOT homologous protein; note (original language) = TOT同源蛋白
MDTVRELNGGSGSPGIPLSLITAAVGAIIILSLLLLRRSKRGNSSHPPGNSGLPFIGETLSFTKAFKSNTLDQFFEERVKKFGQVFKLSVIGPPTVAMCGPEGNRFVFANEEKLVHLSWSGRYAKILGGDSVSMKRGDDHRRVRAAFAGFLSPASLPVYISKMSAQIQDHINEKWKEKVVIAVVPLVKELVFNVSYNLFFSINDSEELHRLHKIFETIVEGHVSMPIDLPGFTFHRALQGRAKLKKVFSSLIERRRSDLSSGLASANQDLISVLLTYKDDRGYTMTHDELLDNFLSLLESSYDSVNSPMACIFKLLYDNPECYEKVVQEQLGILSGKKEGQEISWKDLRSMKYTWQVLQETLRLYTQVAGIFRKAMTDIHYDGHTIPKGWQLLWATQTTHLNDKYFSEPEKFMPSRFDEEGNNLIPYSFVPFGGGRRMCPGWEFGKMEILLFVHHFVKAFSGFTPIDPDEKITGNPFPHLPANGFSIKPTPRS

SEQ ID NO: 33 - protein, 493 aa, unidentified
  source 1..493: note = TOT homologous protein; note (original language) = TOT同源蛋白
MDTVRELNGGSGSPGIPLSLITAAVGAIIILSLLLLRRSKRGNSSHPPGNSGLPFIGETLSFTKAFKSNTLDQFFEERVKKFGQVFKLSVIGPPTVAMCGPEGNRFVFANEEKLVHLSWSGRYAKILGGDSVSMKRGDDHRRVRAAFAGFLSPASLPVYISKMSAQIQDHINEKWKEKVVIAVVPLVKELVFNVSYNLFFSINDSEELHRLHKIFETIVEGHVSMPIDLPGFTFHRALQGRAKLKKVFSSLIERRRSDLSSGLASANQDLISVLLTYKDDRGYTMTHDELLDNFLSLLESSYDSVNSPMACIFKLLYDNPECYEKVVQEQLGILSGKKEGQEISWKDLRSMKYTWQVLQETLRLYTQVAGIFRKAMTDIHYDGHTIPKGWQLLWATQTTHLNDKYFSEPEKFMPSRFDEEGNNLIPYSFVPFGGGRRMCPGWEFGKMEILLFVHHFVKTFSGFTPIDPDEKITGNPFPHLPANGFSIKPTPRS

SEQ ID NO: 34 - protein, 507 aa, unidentified
  source 1..507: note = TOT homologous protein; note (original language) = TOT同源蛋白
MVHVLQVVKMDRVSEIFNGSSGSPAGIPHSVITAGVGAIIIILLSLVLLRRSSKRGDSSHPPGNSGLPFIGETLSFTKAFKSNTLAEFFEERVKKFGNVFKISIIGPPTVVMCGNEGNRFIFANEEKLMHLSWSGRYAKILGGESVSMKRGDDHRSVRAAFAGFLSPSALPLYVAKMSAQIQNHINEKWKGRDVIAVVPLVKELVFNVSSNLFFSMNDSEELHLLHQIFETIVDGHVSMPIDLPGFTFHKALQGRAKLKKVYSSLIERRRSDLSSGLASANQDLISVLLTYKDDRGYTMTHDELLDNFLSLIESSYDSINSPMACIFKLLYANPECYEKVVQEQLGILSGKKEGEEISWKDLRSMKYTWQAIQETLRIYTQVAGIFRKAMTDIHYDGHTIPKGWQLLWATQTTHLNDKYFSEPEKFMPSRFDEEGNNVIPYSFVPFGGGRRMCPGWEFGKMEILLFVHHFVKTFSGFTPIDPNEKITGNPFPHLPANGFLIKPILRS

SEQ ID NO: 35 - protein, 493 aa, unidentified
  source 1..493: note = TOT homologous protein; note (original language) = TOT同源蛋白
MDTVRELNGGSGSPGIPLSLITAAVGAIIILSLLLLRRSKRGNSSHPPGNSGLPFIGETLSFTKAFKSNTLDQFFEERVKKFGQVFKLSVIGPPTVAMCGPEGNRFVFANEEKLVHLSWSGRYAKILGGDSVSMKRGDDHRSVRAAFAGFLSPASLPVYISKMSAQIQDHINEKWKGKDVIAVVPLVKELVFNVSYNLFFSLNDSEELHRLHKIFETIVEGHVSMPIDLPGFTFHRALQGRAKLKKVFSSLIERRRSDLSSGLASANQDLISVLLTYKDDRGYTMTHDELLDNFLSLLEASYDSVNSPMACIFKLLYDNPECYEKVVQEQLGILSGKKEGQEISWKDLRSMKYTWQVLQETLRLYTQVAGIFRKAMTDIHYDGHTIPKGWQLLWATQTTHLNDKYFSEPEKFMPSRFDEEGNNLIPYSFVPFGGGRRMCPGWEFGKMEILLFVHHFVKTFSGFTPIDPDEKITGNPFPHLPANGFSIKPTPRS

SEQ ID NO: 36 - protein, 498 aa, unidentified
  source 1..498: note = TOT homologous protein; note (original language) = TOT同源蛋白
MDRVREIFNGSSGSPAGIPHSVITAGVGAIIIILLSLLLLRRSSKRGDSSHPPGNSGLPFIGETLSFTKAFKSNTLAEFFEERVKKFGNVFKISIIGPPTVVMCGNEGNRFIFANEEKLMHLSWSGRYAKILGGESVSMKRGDDHRSVRAAFAGFLSSASLPVYISKMSAQIQDHINEKWKGKDVIAVVPLVKELVFNVSYNLFFSINDSEELHRLHKIFETIVEGHLSMPIDLPGFTFHRALQGRAKLKKVFSSLIERRRSDLSSGLASANQDLISVLLTYKDDRGYTMTHDELLDNFLSLLEGSYDSINSPMACIFKLLYDNPECYEKVVQEQLGILSGKKEGQEISWKDLRSMKYTWQVLQETLRLYTQVAGIFRKAMTDIHYDGHTIPKGWQLLWANQTTHLNDKYFSEPEKFMPSRFDEEGNNMIPYSFVPFGGGRRMCPGWEFGKMEILLFVHHFVKTFSGFTPIDPNEKITGNPFPHLPANGFLIKPILRS

SEQ ID NO: 37 - protein, 498 aa, unidentified
  source 1..498: note = TOT homologous protein; note (original language) = TOT同源蛋白
MDRVSEIFNGSSGSPAGIPHSVITAGVGAIIIILLSLVLLRRSSKRGDSSHPPGNSGLPFIGETLSFTKAFKSNTLAEFFEERVKKFGNVFKISIIGPPTVVMCGNEGNRFIFANEEKLMHLSWSGRYAKILGGESVSMKRGDDHRSVRAAFAGFLSPSALPLYVAKMSAQIQNHINEKWKGRDVIAVVPLVKELVFNVSSNLFFSMNDSEELHLLHQIFETIVDGHVSMPIDLPGFTFHKALQGRAKLKKVYSSLIERRRSDLSSGLASANQDLISVLLTYKDDRGYTMTHDELLDNFLSLIESSYDSINSPMACIFKLLYANPECYEKVVQEQLGILSGKKEGEEISWKDLRSMKYTWQAIQETLRIYTQVAGIFRKAMTDIHYDGHTIPKGWQLLWATQTTHLNDKYFSEPEKFMPSRFDEEGNNVIPYSFVPFGGGRRMCPGWEFGKMEILLFVHHFVKTFSGFTPIDPNEKITGNPFPHLPANGFLIKPILRS

SEQ ID NO: 38 - protein, 507 aa, unidentified
  source 1..507: note = TOT homologous protein; note (original language) = TOT同源蛋白
MVHVLQVVKMDRVREIFNGSSGSPAGIPHSVITAGVGAIIIILLSLLLLRRSSKRGDSSHPPGNSGLPFIGETLSFTKAFKSNTLAEFFEERVKKFGNVFKISIIGPPTVVMCGNEGNRFIFANEEKLMHLSWSGRYAKILGGESVSMKRGDDHRSVRAAFAGFLSPASLPIYISKMSAQIQDHINKKWKGKDVIAVVPLVKELVFNVSYNLFFSINDSEELHRLHKIFETIVEGHVSMPIDLPGFTFHRALQGRAKLKKVYSSLIERRRSDLSSGLASANQDLISVLLTYKDDRGYRMTHDELLDNFLSLLESSYDSVNSPMACILKLLYANPECYEKVVQEQLGILSGKKEGEEISWKDLRSMKYTWQVLQETLRLYTQVAGIFRKAMTDIHYDGHTIPKGWQLLWATQTTHLNDKYFSEPEKFMPSRFDEEGNNVIPYSFVPFGGGRRMCPGWEFGKMEILLFVHHFVKTFSGFTPIDPNEKITGNPFPHLPANGFLIKPILRS

SEQ ID NO: 39 - protein, 507 aa, unidentified
  source 1..507: note = TOT homologous protein; note (original language) = TOT同源蛋白
MVHVLQVVKMDRVREIFNGSSGSPAGIPHSVITAGVGAIIIILLSLLLLRRSSKRGDSSHPPGNSGLPFIGETLSFTKAFKSNTLAEFFEERVKKFGNVFKISIIGPPTVVMCGNEGNRFIFANEEKLMHLSWSGRYAKILGGESVSMKRGDDHRSVRAAFAGFLSPSALPLYVAKMSAQIQNHINEKWKGRDVIAVVPLVKELVFNVSSNLFFSMNDSEELHRLHQIFETIVDGHVSMPIDLPGFTFHKALQGRAKLKKVYSSLIERRRSDLSSGLASANQDLISVLLTYKDDRGYRMTHDELLDNFLSLLESSYDSVNSPMACILKLLYANPECYEKVVQEQLGILSGKKEGEEISWKDLRSMKYTWQVLQETLRLYTQVAGIFRKAMTDIHYDGHTIPKGWQLLWATQTTHLNDKYFSEPEKFMPSRFDEEGNNVIPYSFVPFGGGRRMCPGWEFGKMEILLFVHHFVKTFSGFTPIDPNEKITGNPFPHLPANGFLIKPILRS

SEQ ID NO: 40 - protein, 498 aa, unidentified
  source 1..498: note = TOT homologous protein; note (original language) = TOT同源蛋白
MDRVREIFNGSSGSPAGIPHSVITAGVGAIIIILLSLLLLRRSSKRGDSSHPPGNSGLPFIGETLSFTKAFKSNTLAEFFEERVKKFGNVFKISIIGPPTVVMCGNEGNRFIFANEEKLMHLSWSGRYAKILGGESVSMKRGDDHRSVRAAFAGFLSPASLPIYISKMSAQIQDHINKKWKGKDVIAVVPLVKELVFNVSYNLFFSINDSEELHRLHKIFETIVEGHVSMPIDLPGFTFHRALQGRAKLKKVYSSLIERRRSDLSSGLASANQDLISVLLTYKDDRGYRMTHDELLDNFLSLLESSYDSVNSPMACILKLLYANPECYEKVVQEQLGILSGKKEGEEISWKDLRSMKYTWQVLQETLRLYTQVAGIFRKAMTDIHYDGHTIPKGWQLLWATQTTHLNDKYFSEPEKFMPSRFDEEGNNVIPYSFVPFGGGRRMCPGWEFGKMEILLFVHHFVKTFSGFTPIDPNEKITGNPFPHLPANGFLIKPILRS

SEQ ID NO: 41 - protein, 498 aa, unidentified
  source 1..498: note = TOT homologous protein; note (original language) = TOT同源蛋白
MDRVREIFNGSSGSPAGIPHSVITAGVGAIIIILLSLLLLRRSSKRGDSSHPPGNSGLPFIGETLSFTKAFKSNTLAEFFEERVKKFGNVFKISIIGPPTVVMCGNEGNRFIFANEEKLMHLSWSGRYAKILGGESVSMKRGDDHRSVRAAFAGFLSPSALPLYVAKMSAQIQNHINEKWKGRDVIAVVPLVKELVFNVSSNLFFSMNDSEELHRLHQIFETIVDGHVSMPIDLPGFTFHKALQGRAKLKKVYSSLIERRRSDLSSGLASANQDLISVLLTYKDDRGYRMTHDELLDNFLSLLESSYDSVNSPMACILKLLYANPECYEKVVQEQLGILSGKKEGEEISWKDLRSMKYTWQVLQETLRLYTQVAGIFRKAMTDIHYDGHTIPKGWQLLWATQTTHLNDKYFSEPEKFMPSRFDEEGNNVIPYSFVPFGGGRRMCPGWEFGKMEILLFVHHFVKTFSGFTPIDPNEKITGNPFPHLPANGFLIKPILRS

SEQ ID NO: 42 - protein, 507 aa, unidentified
  source 1..507: note = TOT homologous protein; note (original language) = TOT同源蛋白
MVHVLQVVKMDRVSEIFNGSSGSPAGIPHSVITAGVGAIIIILLSLLLLRRSSKRGDSSHPPGNSGLPFIGETLSFTKAFKSNTLAEFFEERVKKFGNVFKISIIGPPTVVMCGNEGNRFIFANEEKLMHLSWSGRYAKILGGESVSMKRGDDHRSVRAAFAGFLSPSALPLYVAKMSAQIQNHINEKWKGRDVIAVVPLVKELVFNVSSNLFFSMNDSEELHRLHQIFETIVDGHVSMPIDLPGFTFHKALQGRAKLKKVYSSLIERRRSDLSSGLASANQDLISVLLTYKDDRGYTMTHDELLDNFLSLIESSYDSINSPMACIFKLLYANPECYEKVVQEQLGILSGKKEGEEISWKDLRSMKYTWQAIQETLRIYTQVAGIFRKAMTDIHYDGHTIPKGWQLLWATQTTHLNDKYFSEPEKFMPSRFDEEGNNVIPYSFVPFGGGRRMCPGWEFGKMEILLFVHHFVKTFSGFTPIDPNEKITGNPFPHLPANGFLIKPILRS

SEQ ID NO: 43 - protein, 497 aa, unidentified
  source 1..497: note = TOT homologous protein; note (original language) = TOT同源蛋白
MDVFYPLKSAVTKFNECFPAILFIVLSAVAGIVLPLLLFLRSKRRSSVGLPPGKLGYPFIGESLLFLKALRSNTVEQFLDERVKKFGNVFKTSLIGHPTVVLCGPAGNRLILANEEKLVQMSWPKSSMKLMGEKSITAKRGEGHMIIRSALQGFFSPGALQKYIGQMSKTIENHINEKWKGNDQVSVVALVGDLVFDISACLFFNINEKHERERLFELLEIIAVGVLAVPVDLPGFAYRRALQARSKLNAILSGLIEKRKMDLSSGLASSNQDLLSVFLTFKDDRGNPLSDEEILDNFSGLLHGSYDTTVSAMACVFKLLSSNPECYEKVVQEQLGILSGKKEGQEISWKDLRSMKYTWQVLQETLRLYTQVAGIFRKAMTDIHYDGHTIPKGWQLLWATQTTHLNDKYFSEPEKFMPSRFDEEGNNVIPYSFVPFGGGRRMCPGWEFGKMEILLFVHHFVKAFSGFTPIDPDEKITGNPFPHLPANGFLIKPILRS

SEQ ID NO: 44 - protein, 498 aa, unidentified
  source 1..498: note = TOT homologous protein; note (original language) = TOT同源蛋白
MDRVSEIFNGSSGSPAGIPHSVITAGVGAIIIILLSLLLLRRSSKRGDSSHPPGNSGLPFIGETLSFTKAFKSNTLAEFFEERVKKFGNVFKISIIGPPTVVMCGNEGNRFIFANEEKLMHLSWSGRYAKILGGESVSMKRGDDHRSVRAAFAGFLSPSALPLYVAKMSAQIQNHINEKWKGRDVIAVVPLVKELVFNVSSNLFFSMNDSEELHRLHQIFETIVDGHVSMPIDLPGFTFHKALQGRAKLKKVYSSLIERRRSDLSSGLASANQDLISVLLTYKDDRGYTMTHDELLDNFLSLIESSYDSINSPMACIFKLLYANPECYEKVVQEQLGILSGKKEGEEISWKDLRSMKYTWQAIQETLRIYTQVAGIFRKAMTDIHYDGHTIPKGWQLLWATQTTHLNDKYFSEPEKFMPSRFDEEGNNVIPYSFVPFGGGRRMCPGWEFGKMEILLFVHHFVKTFSGFTPIDPNEKITGNPFPHLPANGFLIKPILRS

SEQ ID NO: 45 - protein, 507 aa, unidentified
  source 1..507: note = TOT homologous protein; note (original language) = TOT同源蛋白
MVHVLQVVKMDRVNEIFNGSSGSPAGIPHSVITAGVGAIIIILLSLLLLRRSSKRGDSAHPPGNSGLPFIGETLSFTKAFKSNTLAEFFEERVKKFGNVFKISIIGPPTVVMCGNEGNRFIFANEEKLMHLSWSGRYAKILGGESVSMKRGDDHRSVRAAFAGFLSSASLPVYISKMSAQIQDHINEKWKGKDVIAVVPLVKELVFNVSYNLFFSINDSEELHRLHKIFETIVEGHVSMPIDLPGFTFHRALQGREKLKKVFSSLIERRRSDLSSGLASANQDLISVLLTYKDDRGYTMTHDELLDNFLSLLESSYDSVNSPMACIFKLLYDNPECYEKVVQEQLGILSGKKEGQEISWKDLRSMKYTWQVLQETLRLYTQVAGIFRKAMTDIHYDGHTIPKGWQLLWATQTTHLNDKYFSEPEKFMPSRFGEEGNNLIPYSFVPFGGGRRMCPGWEFGKMEILLFVHHFVKTFSGFTPIDPDEKITGNPFPHLPANGFSIKPTPRS

SEQ ID NO: 46 - protein, 498 aa, unidentified
  source 1..498: note = TOT homologous protein; note (original language) = TOT同源蛋白
MDRVNEIFNGSSGSPAGIPHSVITAGVGAIIIILLSLLLLRRSSKRGDSAHPPGNSGLPFIGETLSFTKAFKSNTLAEFFEERVKKFGNVFKISIIGPPTVVMCGNEGNRFIFANEEKLMHLSWSGRYAKILGGESVSMKRGDDHRSVRAAFAGFLSSASLPVYISKMSAQIQDHINEKWKGKDVIAVVPLVKELVFNVSYNLFFSINDSEELHRLHKIFETIVEGHVSMPIDLPGFTFHRALQGREKLKKVFSSLIERRRSDLSSGLASANQDLISVLLTYKDDRGYTMTHDELLDNFLSLLESSYDSVNSPMACIFKLLYDNPECYEKVVQEQLGILSGKKEGQEISWKDLRSMKYTWQVLQETLRLYTQVAGIFRKAMTDIHYDGHTIPKGWQLLWATQTTHLNDKYFSEPEKFMPSRFGEEGNNLIPYSFVPFGGGRRMCPGWEFGKMEILLFVHHFVKTFSGFTPIDPDEKITGNPFPHLPANGFSIKPTPRS

SEQ ID NO: 47 - protein, 507 aa, unidentified
  source 1..507: note = TOT homologous protein; note (original language) = TOT同源蛋白
MVHVLQVVKMDRVSEIFNGSSGSPAGIPHSVITAGVGAIIIILLSLVLLRRSSKRGDSSHPPGNSGLPFIGETLSFTKAFKSNTLAEFFEERVKKFGNVFKISIIGPPTVVMCGNEGNRFIFANEEKLMHLSWSGRYAKILGGESVSMKRGDDHRSVRAAFAGFLSPSALPLYVAKMSAQIQNHINEKWKGRDVIAVVPLVKELVFNVSSNLFFGMNDSEELHRLHQIFETIVDGHVSMPIDLPGFTFHKALQGRAKLKKVYSSLIERRRSDLSSGLASANQDLISVLLTYKDDRGYTMTHVELLDNFLSLIESSYDSINSPMACIFKLLYANPECYEKVVQEQLGILSGKKKGEEISWKDLRSMKYTWQAIQETLRIYTQVAGIFRKAMTDIHYDGHTIPKGWQLLWATQTTHLNDKYFSEPEKFMPSRFDEEGNNVIPYSFVPFGGGRRMCPGWEFGKMEILLFVHHFVKTFSGFTPIDPNEKITGNPFPHLPANGFLIKPILRS

SEQ ID NO: 48 - protein, 510 aa, unidentified
  source 1..510: note = TOT homologous protein; note (original language) = TOT同源蛋白
MDSLHRVIKISAIFNGDTKLHWSSPAVFSVAFTAVAGILLLLLLLRSKRRHSSLNQYNLPRGNSGLPFVGETISFLRAFRGNRIQQFFDERAKKFGNVFRISITGPPTAVLCGSEGNRFILSNEEKLVRVDMSGAFSKLAGRDSVMMRTGEEHRTIRAAMAGFLAPTALPIYVGKMSAQIQNHIDEKWKGKDVVTVVSLVKELVFGVSASMFYDINDGVEQHRLHEIYQTMVAGHFSFPLDFPGFSFHRAVQGRQKLKKIFSSLIEKRRSDLRSGLASSNQDLLSVLLTYKNEKGNGLTQGELTDNFITMLEASYDNPVSAISCILKFLYSHPEVYEKVVQEQLGILSNKEEGDEISWKDVKAMKYTWQAVQETLRMISPVIGILRKAMTDIHYDGYTIPKGWQLLWTGCSTHLKDAYFNEADEFMPSRFDEEGKNVVPYSFVPFGGGRRMCPGWEFSKLAILLFVHHFVKTFSSYTPLDPDEKILGNPFPLLPVNGLSIKLTARSEIKN

SEQ ID NO: 49 - DNA, 42 bp, synthetic construct
  source 1..42: mol_type = other DNA; note = P1
gtatattctgcccaaattcgcgaatggttcatgtgttgcagg

SEQ ID NO: 50 - DNA, 53 bp, synthetic construct
  source 1..53: mol_type = other DNA; note = P2
accagagttaaaggcctcgagttaggatctgggagtaggttttattgaaaatc

SEQ ID NO: 51 - DNA, 44 bp, synthetic construct
  source 1..44: mol_type = other DNA; note = P3
gtcaaggagaaaaaaccccggatccatggttcatgtgttgcagg

SEQ ID NO: 52 - DNA, 48 bp, synthetic construct
  source 1..48: mol_type = other DNA; note = P4
aaatcaacttctgttccatgtcgacggatctgggagtaggttttattg

SEQ ID NO: 53 - DNA, 54 bp, synthetic construct
  source 1..54: mol_type = other DNA; note = P5
ttcaaaggcctacgtcgacgagctcatggttcatgtgttgcaggtagtgaaaat

SEQ ID NO: 54 - DNA, 79 bp, synthetic construct
  source 1..79: mol_type = other DNA; note = P6
caggctctagattcgaaagcggccgcctagtgatggtgatggtgatgggatctgggagtaggttttattgaaaatccat

SEQ ID NO: 55 - DNA, 48 bp, synthetic construct
  source 1..48: mol_type = other DNA; note = P7
ttcaaaggcctacgtcgacgagctcatgcaggctaattccaacacggt

SEQ ID NO: 56 - DNA, 81 bp, synthetic construct
  source 1..81: mol_type = other DNA; note = P8
caggctctagattcgaaagcggccgctcagtgatggtgatggtgatgccatatatctcgtaagtatcttccatccatctgt

SEQ ID NO: 57 - DNA, 43 bp, synthetic construct
  source 1..43: mol_type = other DNA; note = P9
gtatattctgcccaaattcgcgaatggttcatgtgttgcaggt

SEQ ID NO: 58 - DNA, 54 bp, synthetic construct
  source 1..54: mol_type = other DNA; note = P10
accagagttaaaggcctcgagttaggatctgagaataggttttattagaaatcc

SEQ ID NO: 59 - DNA, 42 bp, synthetic construct
  source 1..42: mol_type = other DNA; note = P11
gtatattctgcccaaattcgcgaatggttcatgtgttgcacg

SEQ ID NO: 60 - DNA, 58 bp, synthetic construct
  source 1..58: mol_type = other DNA; note = P12
accagagttaaaggcctcgagttaggatctgagaataggttttattagaaatccattg

SEQ ID NO: 61 - DNA, 43 bp, synthetic construct; identical to SEQ ID NO: 57
  source 1..43: mol_type = other DNA; note = P13

SEQ ID NO: 62 - DNA, 58 bp, synthetic construct; identical to SEQ ID NO: 60
  source 1..58: mol_type = other DNA; note = P14

SEQ ID NO: 63 - DNA, 59 bp, synthetic construct
  source 1..59: mol_type = other DNA; note = Q6A-F
tcatgtgttggctgtagtgaaaatggatagagttagagaaatatttaatggaagttcag

SEQ ID NO: 64 - DNA, 39 bp, synthetic construct
  source 1..39: mol_type = other DNA; note = Q6A-R
ttttcactacagccaacacatgaaccattcgcgaatttg

SEQ ID NO: 65 - DNA, 35 bp, synthetic construct
  source 1..35: mol_type = other DNA; note = F122A-F
ccggtttattgctgccaacgaggagaagcttgtcc

SEQ ID NO: 66 - DNA, 37 bp, synthetic construct
  source 1..37: mol_type = other DNA; note = F122A-R
cctcgttggcagcaataaaccggtttccctcattgcc

SEQ ID NO: 67 - DNA, 38 bp, synthetic construct
  source 1..38: mol_type = other DNA; note = V129A-F
ggagaagcttgctcacttgtcgtggtctggtcgatatg

SEQ ID NO: 68 - DNA, 41 bp, synthetic construct
  source 1..41: mol_type = other DNA; note = V129A-R
acgacaagtgagcaagcttctcctcgttggcgaaaataaac

SEQ ID NO: 69 - DNA, 34 bp, synthetic construct
  source 1..34: mol_type = other DNA; note = L131A-F
gcttgtccacgcttcgtggtctggtcgatatgcg

SEQ ID NO: 70 - DNA, 36 bp, synthetic construct
  source 1..36: mol_type = other DNA; note = L131A-R
cagaccacgaagcgtggacaagcttctcctcgttgg

SEQ ID NO: 71 - DNA, 38 bp, synthetic construct
  source 1..38: mol_type = other DNA; note = W133A-F
ccacttgtcggcttctggtcgatatgcgaaaatcctgg

SEQ ID NO: 72 - DNA, 35 bp, synthetic construct
  source 1..35: mol_type = other DNA; note = W133A-R
atcgaccagaagccgacaagtggacaagcttctcc

SEQ ID NO: 73 - DNA, 36 bp, synthetic construct
  source 1..36: mol_type = other DNA; note = Y137A-F
gtctggtcgagctgcgaaaatcctgggtggagattc

SEQ ID NO: 74 - DNA, 34 bp, synthetic construct
  source 1..34: mol_type = other DNA; note = Y137A-R
ggattttcgcagctcgaccagaccacgacaagtg

SEQ ID NO: 75 - DNA, 38 bp, synthetic construct
  source 1..38: mol_type = other DNA; note = D144A-F
cctgggtggagcttccgtttccatgaagaggggagatg

SEQ ID NO: 76 - DNA, 39 bp, synthetic construct
  source 1..39: mol_type = other DNA; note = D144A-R
tggaaacggaagctccacccaggattttcgcatatcgac

SEQ ID NO: 77 - DNA, 39 bp, synthetic construct
  source 1..39: mol_type = other DNA; note = V146A-F
tggagattccgcttccatgaagaggggagatgatcatcg

SEQ ID NO: 78 - DNA, 37 bp, synthetic construct
  source 1..37: mol_type = other DNA; note = V146A-R
tcttcatggaagcggaatctccacccaggattttcgc

SEQ ID NO: 79 - DNA, 37 bp, synthetic construct
  source 1..37: mol_type = other DNA; note = S147A-F
agattccgttgctatgaagaggggagatgatcatcgc

SEQ ID NO: 80 - DNA, 32 bp, synthetic construct
  source 1..32: mol_type = other DNA; note = S147A-R
ccctcttcatagcaacggaatctccacccagg

SEQ ID NO: 81 - DNA, 29 bp, synthetic construct
  source 1..29: mol_type = other DNA; note = H154A-F
gggagatgatgctcgcagtgtacgtgccg

SEQ ID NO: 82 - DNA, 38 bp, synthetic construct
  source 1..38: mol_type = other DNA; note = H154A-R
gtacactgcgagcatcatctcccctcttcatggaaacg

SEQ ID NO: 83 - DNA, 29 bp, synthetic construct
  source 1..29: mol_type = other DNA; note = R158A-F
tcgcagtgtagctgccgcattcgcagggt

SEQ ID NO: 84 - DNA, 38 bp, synthetic construct
  source 1..38: mol_type = other DNA; note = R158A-R
cgaatgcggcagctacactgcgatgatcatctcccctc

SEQ ID NO: 85 - DNA, 47 bp, synthetic construct
  source 1..47: mol_type = other DNA; note = P167A-F
gtttttgagcgctgcatcgctgcctatttacataagtaaaatgagtg

SEQ ID NO: 86 - DNA, 35 bp, synthetic construct
  source 1..35: mol_type = other DNA; note = P167A-R
gcagcgatgcagcgctcaaaaaccctgcgaatgcg

SEQ ID NO: 87 - DNA, 52 bp, synthetic construct
  source 1..52: mol_type = other DNA; note = I172A-F
atcgctgcctgcttacataagtaaaatgagtgcacagatccaagatcatatc

SEQ ID NO: 88 - DNA, 30 bp, synthetic construct
  source 1..30: mol_type = other DNA; note = I172A-R
tacttatgtaagcaggcagcgatgcagggc

SEQ ID NO: 89 - DNA, 48 bp, synthetic construct
  source 1..48: mol_type = other DNA; note = Q187A-F
tcatatcaacgctaaatggaaaggaaaagatgtaattgctgtagttcc

SEQ ID NO: 90 - DNA, 48 bp, synthetic construct
  source 1..48: mol_type = other DNA; note = Q187A-R
ctttccatttagcgttgatatgatcttggatctgtgcactcattttac

SEQ ID NO: 91 - DNA, 35 bp, synthetic construct
  source 1..35: mol_type = other DNA; note = V237A-F
ggagggacatgcttccatgccgatagaccttcccg

SEQ ID NO: 92 - DNA, 46 bp, synthetic construct
  source 1..46: mol_type = other DNA; note = V237A-R
tcggcatggaagcatgtccctccacaatagtttcgaaaatcttatg

SEQ ID NO: 93 - DNA, 43 bp, synthetic construct
  source 1..43: mol_type = other DNA; note = S310A-F
caactttcttgctcttcttgaatcctcctatgattccgtcaat

SEQ ID NO: 94 - DNA, 36 bp, synthetic construct
  source 1..36: mol_type = other DNA; note = S310A-R
attcaagaagagcaagaaagttgtcgaggagctcgt

SEQ ID NO: 95 - DNA, 39 bp, synthetic construct
  source 1..39: mol_type = other DNA; note = E313A-F
ttcccttcttgcttcctcctatgattccgtcaattcacc

SEQ ID NO: 96 - DNA, 40 bp, synthetic construct
  source 1..40: mol_type = other DNA; note = E313A-R
cataggaggaagcaagaagggaaagaaagttgtcgaggag

SEQ ID NO: 97 - DNA, 42 bp, synthetic construct
  source 1..42: mol_type = other DNA; note = S314A-F
ccttcttgaagcttcctatgattccgtcaattcaccaatggc

SEQ ID NO: 98 - DNA, 41 bp, synthetic construct
  source 1..41: mol_type = other DNA; note = S314A-R
aatcataggaagcttcaagaagggaaagaaagttgtcgagg

SEQ ID NO: 99 - DNA, 36 bp, synthetic construct
  source 1..36: mol_type = other DNA; note = S318A-F
ctcctatgatgctgtcaattcaccaatggcctgcat

SEQ ID NO: 100 - DNA, 44 bp, synthetic construct
  source 1..44: mol_type = other DNA; note = S318A-R
gtgaattgacagcatcataggaggattcaagaagggaaagaaag

SEQ ID NO: 101 - DNA, 41 bp, synthetic construct
  source 1..41: mol_type = other DNA; note = V319A-F
ctatgattccgctaattcaccaatggcctgcatttttaagc

SEQ ID NO: 102 - DNA, 43 bp, synthetic construct
  source 1..43: mol_type = other DNA; note = V319A-R
ttggtgaattagcggaatcataggaggattcaagaagggaaag

SEQ ID NO: 103 - DNA, 44 bp, synthetic construct
  source 1..44: mol_type = other DNA; note = L330A-F
ttttaagcttgcttatgccaatccagaatgctatgaaaaagtag

SEQ ID NO: 104 - DNA, 37 bp, synthetic construct
  source 1..37: mol_type = other DNA; note = L330A-R
gattggcataagcaagcttaaaaatgcaggccattgg

SEQ ID NO: 105 - DNA, 44 bp, synthetic construct
  source 1..44: mol_type = other DNA; note = I347A-F
gcaattgggggctctttctggtaagaaggaaggacaagaaatct

SEQ ID NO: 106 - DNA, 42 bp, synthetic construct
  source 1..42: mol_type = other DNA; note = I347A-R
taccagaaagagcccccaattgctcttgaactactttttcat

SEQ ID NO: 107 - DNA, 41 bp, synthetic construct
  source 1..41: mol_type = other DNA; note = D361A-F
ctcgtggaaggctctgagatccatgaaatacacatggcaag

SEQ ID NO: 108 - DNA, 39 bp, synthetic construct
  source 1..39: mol_type = other DNA; note = D361A-R
tggatctcagagccttccacgagatttcttgtccttcct

SEQ ID NO: 109 - DNA, 43 bp, synthetic construct
  source 1..43: mol_type = other DNA; note = M365A-F
tctgagatccgctaaatacacatggcaagtacttcaggaaacg

SEQ ID NO: 110 - DNA, 40 bp, synthetic construct
  source 1..40: mol_type = other DNA; note = M365A-R
atgtgtatttagcggatctcagatccttccacgagatttc

SEQ ID NO: 111 - DNA, 37 bp, synthetic construct
  source 1..37: mol_type = other DNA; note = Y367A-F
atccatgaaagctacatggcaagtacttcaggaaacg

SEQ ID NO: 112 - DNA, 39 bp, synthetic construct
  source 1..39: mol_type = other DNA; note = Y367A-R
cttgccatgtagctttcatggatctcagatccttccacg

SEQ ID NO: 113 - DNA, 40 bp, synthetic construct
  source 1..40: mol_type = other DNA; note = V371A-F
cacatggcaagctcttcaggaaacgctacgactgtatact

SEQ ID NO: 114 - DNA, 43 bp, synthetic construct
  source 1..43: mol_type = other DNA; note = V371A-R
tttcctgaagagcttgccatgtgtatttcatggatctcagatc

SEQ ID NO: 115 - DNA, 43 bp, synthetic construct
  source 1..43: mol_type = other DNA; note = R377A-F
ggaaacgctagctctgtatactcaagttgctggaatatttcgc

SEQ ID NO: 116 - DNA, 39 bp, synthetic construct
  source 1..39: mol_type = other DNA; note = R377A-R
gagtatacagagctagcgtttcctgaagtacttgccatg

SEQ ID NO: 117 - DNA, 37 bp, synthetic construct
  source 1..37: mol_type = other DNA; note = Q381A-F
actgtatactgctgttgctggaatatttcgcaaagcc

SEQ ID NO: 118 - DNA, 40 bp, synthetic construct
  source 1..40: mol_type = other DNA; note = Q381A-R
ttccagcaacagcagtatacagtcgtagcgtttcctgaag

SEQ ID NO: 119 - DNA, 37 bp, synthetic construct
  source 1..37: mol_type = other DNA; note = V382A-F
gtatactcaagctgctggaatatttcgcaaagccatg

SEQ ID NO: 120 - DNA, 40 bp, synthetic construct
  source 1..40: mol_type = other DNA; note = V382A-R
atattccagcagcttgagtatacagtcgtagcgtttcctg

SEQ ID NO: 121 - DNA, 39 bp, synthetic construct
  source 1..39: mol_type = other DNA; note = G384A-F
tcaagttgctgctatatttcgcaaagccatgactgtcat

SEQ ID NO: 122 - DNA, 39 bp, synthetic construct
  source 1..39: mol_type = other DNA; note = G384A-R
tgcgaaatatagcagcaacttgagtatacagtcgtagcg

SEQ ID NO: 123 - DNA, 38 bp, synthetic construct
  source 1..38: mol_type = other DNA; note = I385A-F
agttgctggagcttttcgcaaagccatgactgtcattc

SEQ ID NO: 124 - DNA, 41 bp, synthetic construct
  source 1..41: mol_type = other DNA; note = I385A-R
ctttgcgaaaagctccagcaacttgagtatacagtcgtagc

SEQ ID NO: 125 - DNA, 42 bp, synthetic construct
  source 1..42: mol_type = other DNA; note = R387A-F
tggaatatttgctaaagccatgactgtcattcattatgatgg

SEQ ID NO: 126 - DNA, 44 bp, synthetic construct
  source 1..44: mol_type = other DNA; note = R387A-R
tcatggctttagcaaatattccagcaacttgagtatacagtcgt

SEQ ID NO: 127 - DNA, 33 bp, synthetic construct
  source 1..33: mol_type = other DNA; note = I400A-F
tggtcacaccgctcccaaagggtggcaacttct

SEQ ID NO: 128 - DNA, 43 bp, synthetic construct
  source 1..43: mol_type = other DNA; note = I400A-R
accctttgggagcggtgtgaccatcataatgaatgacagtcat

SEQ ID NO: 129 - DNA, 37 bp, synthetic construct
  source 1..37: mol_type = other DNA; note = W404A-F
tcccaaaggggctcaacttctttgggcaacccaaact

SEQ ID NO: 130 - DNA, 34 bp, synthetic construct
  source 1..34: mol_type = other DNA; note = W404A-R
aaagaagttgagcccctttgggaatggtgtgacc

SEQ ID NO: 131 - DNA, 47 bp, synthetic construct
  source 1..47: mol_type = other DNA; note = T410A-F
tctttgggcagctcaaactacacatctgaacgacaaatatttcagtg

SEQ ID NO: 132 - DNA, 34 bp, synthetic construct
  source 1..34: mol_type = other DNA; note = T410A-R
gtgtagtttgagctgcccaaagaagttgccaccc

SEQ ID NO: 133 - DNA, 39 bp, synthetic construct
  source 1..39: mol_type = other DNA; note = F426A-F
gccggaaaaagctatgccttccagattcgatgaagaagg

SEQ ID NO: 134 - DNA, 41 bp, synthetic construct
  source 1..41: mol_type = other DNA; note = F426A-R
tggaaggcatagctttttccggctcactgaaatatttgtcg

SEQ ID NO: 135 - DNA, 43 bp, synthetic construct
  source 1..43: mol_type = other DNA; note = P428A-F
aaaattcatggcttccagattcgatgaagaaggaaacaatgtg

SEQ ID NO: 136 - DNA, 44 bp, synthetic construct
  source 1..44: mol_type = other DNA; note = P428A-R
cgaatctggaagccatgaatttttccggctcactgaaatatttg

SEQ ID NO: 137 - DNA, 34 bp, synthetic construct
  source 1..34: mol_type = other DNA; note = F443A-F
tccttactcagctgtaccatttggaggagggcgg

SEQ ID NO: 138 - DNA, 46 bp, synthetic construct
  source 1..46: mol_type = other DNA; note = F443A-R
caaatggtacagctgagtaaggaatcacattgtttccttcttcatc

SEQ ID NO: 139 - DNA, 42 bp, synthetic construct
  source 1..42: mol_type = other DNA; note = G455A-F
gatgtgtccagcttgggaattcggaaagatggagatcttact

SEQ ID NO: 140 - DNA, 30 bp, synthetic construct
  source 1..30: mol_type = other DNA; note = G455A-R
cgaattcccaagctggacacatccgccgcc

SEQ ID NO: 141 - DNA, 30 bp, synthetic construct
  source 1..30: mol_type = other DNA; note = P445A-F
ctcattcgtagcttttggaggagggcggcg

SEQ ID NO: 142 - DNA, 46 bp, synthetic construct
  source 1..46: mol_type = other DNA; note = P445A-R
ctcctccaaaagctacgaatgagtaaggaatcacattgtttccttc

SEQ ID NO: 143 - DNA, 30 bp, synthetic construct
  source 1..30: mol_type = other DNA; note = F446A-F
attcgtaccagctggaggagggcggcggat

SEQ ID NO: 144 - DNA, 52 bp, synthetic construct
  source 1..52: mol_type = other DNA; note = F446A-R
gccctcctccagctggtacgaatgagtaaggaatcacattgtttccttcttc

SEQ ID NO: 145 - DNA, 30 bp, synthetic construct
  source 1..30: mol_type = other DNA; note = G447A-F
cgtaccatttgctggagggcggcggatgtg

SEQ ID NO: 146 - DNA, 53 bp, synthetic construct
  source 1..53: mol_type = other DNA; note = G447A-R
gccgccctccagcaaatggtacgaatgagtaaggaatcacattgtttccttct

SEQ ID NO: 147 - DNA, 29 bp, synthetic construct
  source 1..29: mol_type = other DNA; note = G448A-F
accatttggagctgggcggcggatgtgtc

SEQ ID NO: 148 - DNA, 45 bp, synthetic construct
  source 1..45: mol_type = other DNA; note = G448A-R
tccgccgcccagctccaaatggtacgaatgagtaaggaatcacat

SEQ ID NO: 149 - DNA, 32 bp, synthetic construct
  source 1..32: mol_type = other DNA; note = R450A-F
tggaggaggggctcggatgtgtccaggttggg

SEQ ID NO: 150 - DNA, 38 bp, synthetic construct
  source 1..38: mol_type = other DNA; note = R450A-R
gacacatccgagcccctcctccaaatggtacgaatgag

SEQ ID NO: 151 - DNA, 36 bp, synthetic construct
  source 1..36: mol_type = other DNA; note = R451A-F
aggagggcgggctatgtgtccaggttgggaattcgg

SEQ ID NO: 152 - DNA, 34 bp, synthetic construct
  source 1..34: mol_type = other DNA; note = R451A-R
ctggacacatagcccgccctcctccaaatggtac

SEQ ID NO: 153 - DNA, 37 bp, synthetic construct
  source 1..37: mol_type = other DNA; note = M452A-F
agggcggcgggcttgtccaggttgggaattcggaaag

SEQ ID NO: 154 - DNA, 28 bp, synthetic construct
  source 1..28: mol_type = other DNA; note = M452A-R
aacctggacaagcccgccgccctcctcc

SEQ ID NO: 155 - DNA, 39 bp, synthetic construct
  source 1..39: mol_type = other DNA; note = P454A-F
gcggatgtgtgctggttgggaattcggaaagatggagat

SEQ ID NO: 156 - DNA, 28 bp, synthetic construct
  source 1..28: mol_type = other DNA; note = P454A-R
attcccaaccagcacacatccgccgccc

SEQ ID NO: 157 - DNA, 36 bp, synthetic construct
  source 1..36: mol_type = other DNA; note = P490A-F
tactgggaatgcttttcctcatctccctgccaatgg

SEQ ID NO: 158 - DNA, 40 bp, synthetic construct
  source 1..40: mol_type = other DNA; note = P490A-R
gatgaggaaaagcattcccagtaattttttcgtccggatc

SEQ ID NO: 159 - DNA, 33 bp, synthetic construct
  source 1..33: mol_type = other DNA; note = F491A-F
tgggaatccagctcctcatctccctgccaatgg

SEQ ID NO: 160 - DNA, 40 bp, synthetic construct
  source 1..40: mol_type = other DNA; note = F491A-R
ggagatgaggagctggattcccagtaattttttcgtccgg

SEQ ID NO: 161 - DNA, 39 bp, synthetic construct
  source 1..39: mol_type = other DNA; note = P492A-F
gaatccatttgctcatctccctgccaatggattttcaat

SEQ ID NO: 162 - DNA, 42 bp, synthetic construct
  source 1..42: mol_type = other DNA; note = P492A-R
cagggagatgagcaaatggattcccagtaattttttcgtccg

SEQ ID NO: 163 - DNA, 43 bp, synthetic construct
  source 1..43: mol_type = other DNA; note = S500A-F
caatggatttgctataaaacctactcccagatcctaactcgag

SEQ ID NO: 164 - DNA, 37 bp, synthetic construct
  source 1..37: mol_type = other DNA; note = S500A-R
taggttttatagcaaatccattggcagggagatgagg